European Patent Application EP 4 269 427 A2, published November 1, 2023. Title: Protein Interfaces. Applicant: Synthex, Inc. Application EP. The sequence listing filed with the application follows.

SEQUENCE LISTING (144 sequences)

SEQ ID NO: 1 - protein, 29 aa, synthetic construct
  REGION 1..29: note = Description of Artificial Sequence: Synthetic peptide
KQSLRLGLSRLARVKRLHPGARRRRRRRR

SEQ ID NO: 2 - protein, 29 aa, synthetic construct
  REGION 1..29: note = Description of Artificial Sequence: Synthetic peptide
KQSLRLGQSRLARVKRLHPGARRRRRRRR

SEQ ID NO: 3 - protein, 29 aa, synthetic construct
  REGION 1..29: note = Description of Artificial Sequence: Synthetic peptide
KQSLRLGLSRLARVKRLHPGARRRRRRRR

SEQ ID NO: 4 - protein, 31 aa, synthetic construct
  REGION 1..31: note = Description of Artificial Sequence: Synthetic peptide
KQSNLRLGLSRLARVKRLHPGCCRRRRRRRR

SEQ ID NO: 5 - protein, 21 aa, synthetic construct
  REGION 1..21: note = Description of Artificial Sequence: Synthetic peptide
KRRRRRRRKRLGVRLRVSRML

SEQ ID NO: 6 - protein, 21 aa, synthetic construct
  REGION 1..21: note = Description of Artificial Sequence: Synthetic peptide
KRRRRRRRKRLGQRLRQSRML

SEQ ID NO: 7 - protein, 16 aa, synthetic construct
  REGION 1..16: note = Description of Artificial Sequence: Synthetic peptide
KRRRRRRRRLGMSRRF

SEQ ID NO: 8 - skipped

SEQ ID NO: 9 - protein, 21 aa, synthetic construct
  REGION 1..21: note = Description of Artificial Sequence: Synthetic peptide
KRRRRRRRKRLGLRLGVSRRV

SEQ ID NO: 10 - protein, 20 aa, synthetic construct
  REGION 1..20: note = Description of Artificial Sequence: Synthetic peptide
LMRSVRLRVGLRKRRRRRRR

SEQ ID NO: 11 - protein, 26 aa, synthetic construct
  REGION 1..26: note = Description of Artificial Sequence: Synthetic peptide
KRRRRRRRSLRLGLSRLARVKRLHPG

SEQ ID NO: 12 - skipped

SEQ ID NO: 13 - protein, 13 aa, Human immunodeficiency virus 1
GRKKRRQRRRPPQ

SEQ ID NO: 14 - protein, 8 aa, synthetic construct
  REGION 1..8: note = Description of Artificial Sequence: Synthetic peptide
RRRRRRRR

SEQ ID NO: 15 - protein, 18 aa, unidentified
  REGION 1..18: note = Description of Unknown: MAP sequence
KLALKLALKALKAALKLA

SEQ ID NO: 16 - protein, 27 aa, unidentified
  REGION 1..27: note = Description of Unknown: Transportan sequence
GWTLNSAGYLLGKINLKALAALAKKIL

SEQ ID NO: 17 - protein, 18 aa, unidentified
  REGION 1..18: note = Description of Unknown: Pegelin sequence
RGGRLSYSRRRFSTSTGR

SEQ ID NO: 18 - protein, 16 aa, Drosophila sp.
RQIKIWFQNRRMKWKK

SEQ ID NO: 19 - protein, 8 aa, synthetic construct
  MOD_RES 4: note = Leu, Met or Val
  MOD_RES 7: note = Arg, Leu or Lys
  MOD_RES 8: note = Arg, Phe or Val
  REGION 1..8: note = Description of Artificial Sequence: Synthetic peptide
RLGXSRXX

SEQ ID NO: 20 - protein, 258 aa, Vibrio cholerae
MVKIIFVFFIFLSSFSYANDDKLYRADSRPPDEIKQSGGLMPRGQSEYFDRGTQMNINLYDHARGTQTGFVRHDDGYVSTSISLRSAHLVGQTILSGHSTYYIYVIATAPNMFNVNDVLGAYSPHPDEQEVSALGGIPYSQIYGWYRVHFGVLDEQLHRNRGYRDRYYSNLDIAPAADGYGLAGFPPEHRAWREEPWIHHAPPGCGNAPRSSMSNTCDEKTQSLGVKFLDEYQSKVKRQIFSGYQSDIDTHNRIKDEL

SEQ ID NO: 21 - protein, 593 aa, Salmonella enterica
MLILNGFSSATLALITPPFLPKGGKALSQSGPDGLASITLPLPISAERGFAPALALHYSSGGGNGPFGVGWSCATMSIARRTSHGVPQYNDSDEFLGPDGEVLVQTLSTGDAPNPVTCFAYGDVSFPQSYTVTRYQPRTESSFYRLEYWVGNSNGDDFWLLHDSNGILHLLGKTAAARLSDPQAASHTAQWLVEESVTPAGEHIYYSYLAENGDNVDLNGNEAGRDRSAMRYLSKVQYGNATPAADLYLWTSATPAVQWLFTLVFDYGERGVDPQVPPAFTAQNSWLARQDPFSLYNYGFEIRLHRLCRQVLMFHHFPDELGEADTLVSRLLLEYDENPILTQLCAARTLAYEGDGYRRAPVNNMMPPPPPPPPPMMGGNSSRPKSKWAIVEESKQIQALRYYSAQGYSVINKYLRGDDYPETQAKETLLSRDYLSTNEPSDEEFKNAMSVYINDIAEGLSSLPETDHRVVYRGLKLDKPALSDVLKEYTTIGNIIIDKAFMSTSPDKAWINDTILNIYLEKGHKGRILGDVAHFKGEAEMLFPPNTKLKIESIVNCGSQDFASQLSKLRLSDDATADTNRIKRIINMRVLNS

SEQ ID NO: 22 - protein, 601 aa, Mycoplasma pneumoniae
MSENLYFQGHMPNPVRFVYRVDLRSPEEIFEHGFSTLGDVRNFFEHILSTNFGRSYFISTSETPTAAIRFFGSWLREYVPEHPRRAYLYEIRADQHFYNARATGENLLDLMRQRQVVFDSGDREMAQMGIRALRTSFAYQREWFTDGPIAAANVRSAWLVDAVPVEPGHAHHPAGRVVETTRINEPEMHNPHYQELQTQANDQPWLPTPGIATPVHLSIPQAASVADVSEGTSASLSFACPDWSPPSSNGENPLDKCIAEKIDNYNLQSLPQYASSVKELEDTPVYLRGIKTQKTFMLQADPQNNNVFLVEVNPKQKSSFPQTIFFWDVYQRICLKDLTGAQISLSLTAFTTQYAGQLKVHLSVSAVNAVNQKWKMTPQDIAITQFRVSSELLGQTENGLFWNTKSGGSQHDLYVCPLKNPPSDLEELQIIVDECTTHAQFVTMRAASTFFVDVQLGWYWRGYYYTPQLSGWSYQMKTPDGQIFYDLKTSKIFFVQDNQNVFFLHNKLNKQTGYSWDWVEWLKHDMNEDKDENFKWYFSRDDLTIPSVEGLNFRHIRCYADNQQLKVIISGSRWGGWYSTYDKVESNVEDKILVKDGFDRF

SEQ ID NO: 23 - protein, 250 aa, Streptococcus pyogenes
MLKKRYQLAMILLLSCFSLVWQTEGLVELFVCEHYERAVCEGTPAYFTFSDQKGAETLIKKRWGKGLVYPRAEQEAMAAYTCQQAGPINTSLDKAKGKLSQLTPELRDQVAQLDAATHRLVIPWNIVVYRYVYETFLRDIGVSHADLTSYYRNHQFNPHILCKIKLGTRYTKHSFMSTTALKNGAMTHRPVEVRICVKKGAKAAFVEPYSAVPSEVELLFPRGCQLEVVGAYVSQDHKKLHIEAYFKGSL

SEQ ID NO: 24 - protein, 264 aa, Pseudomonas syringae
MNINRQLPVSGSERLLTPDVGVSRQACSERHYSTGQDRHDFYRFAARLHVDAQCFGLSIDDLMDKFSDKHFRAEHPEYRDVYPEECSAIYMHTAQDYSSHLVRGEIGTPLYREVNNYLRLQHENSGREAEIDNHDEKLSPHIKMLSSALNRLMDVAAFRGTVYRGIRGDLDTIARLYHLFDTGGRYVEPAFMSTTRIKDSAQVFEPGTPNNIAFQISLKRGADISGSSQAPSEEEIMLPMMSEFVIEHASALSEGKHLFVLSQI

SEQ ID NO: 25 - protein, 601 aa, Vibrio cholerae
MKTIISLIFIMFPLFVSAHNGNFYRADSRSPNEIKDLGGLYPRGYYDFFERGTPMSISLYDHARGAPSGNTRYDDGFVSTTTDIDSAHEIGQNILSGYTEYYIYLIAPAPNLLDVNAVLGRYSPHPQENEYSALGGIPWTQVIGWYVVNNGVLDRNIHRNRQFRADLFNNLSPALPSESYQFAGFEPEHPAWRQEPWINFAPPGCGRNVRLTKHINQQDCSNSQEELVYKKLQDLRTQFKVDKKLKLVNKTSSNNIIFPNHDFIREWVDLDGNGDLSYCGFTVDSDGSRKRIVCAHNNGNFTYSSINISLSDYGWPKGQRFIDANGDGLVDYCRVQYVWTHLYCSLSLPGQYFSLDKDAGYLDAGYNNSRAWAKVIGTNKYSFCRLTSNGYICTDIDSYSTAFKDDDQGWADSRYWMDIDGNGGDDYCRLVYNWTHLRCNLQGKDGLWKRVESKYLDGGYPSLRFKIKMTSNKDNYCRIVRNHRVMECAYVSDNGEFHNYSLNMPFSLYNKNDIQFIDIDGDNRDDICRYNSAPNTMECYLNQDKSFSQNKLVLYLSAKPISSLGSGSSKIIRTFNSEKNSSAYCYNAGYGTLRCDEFVIY

SEQ ID NO: 26 - protein, 476 aa, Bacillus cereus
MKEIIRNLVRLDVRSDVDENSKKTQELVEKLPHEVLELYKNVGGEIYITDKRLTQHEELSDSSHKDMFIVSSEGKSFPLREHFVFAKGGKEPSLIIHAEDYASHLSSVEVYYELGKAIIRDTFPLNQKELGNPKFINAINEVNQQKEGKGVNAKADEDGRDLLFGKELKKNLEHGQLVDLDLISGNLSEFQHVFAKSFALYYEPHYKEALKSYAPALFNYMLELDQMRFKEISDDVKEKNKNVLDFKWYTRKAESWGVQTFKNWKENLTISEKDIITGYTGSKYDPINEYLRKYDGEIIPNIGGDLDKKSKKALEKIENQIKNLDAALQKSKITENLIVYRRVSELQFGKKYEDYNLRQNGIINEEKVMELESNFKGQTFIQHNYMSTSLVQDPHQSYSNDRYPILLEITIPEGVHGAYIADMSEYPGQYEMLINRGYTFKYDKFSIVKPTREEDKGKEYLKVNLSIYLGNLNREK

SEQ ID NO: 27 - protein, 487 aa, Enterococcus faecalis V583
MSQLNKWQKELQALQKANYQETDNQLFNVYRQSLIDIKKRLKVYTENAESLSFSTRLEVERLFSVADEINAILQLNSPKVEKTIKGYSAKQAEQGYYGLWYTLEQSQNIALSMPLINHDYIMNLVNAPVAGKRLSKRLYKYRDELAQNVTNNIITGLFEGKSYAEIARWINEETEASYKQALRIARTEAGRTQSVTTQKGYEEAKELGINIKKKWLATIDKHTRRTHQELDGKEVDVDEEFTIRGHSAKGPRMFGVASEDVNCRCTTIEVVDGISPELRKDNESKEMSEFKSYDEWYADRIRQNESKPKPNFTELDFFGQSDLQDDSDKWVAGLKPEQVNAMKDYTSDAFAKMNKILRNEKYNPREKPYLVNIIQNLDDAISKFKLKHDIITYRGVSANEYDAILNGNVFKEFKSTSINKKVAEDFLNFTSANKDGRVVKFLIPKGTQGAYIGTNSSMKKESEFLLNRNLKYTVEIVDNILEVTILG

SEQ ID NO: 28 - protein, 457 aa, Pseudomonas aeruginosa
MHIQSSQQNPSFVAELSQAVAGRLGQVEARQVATPREAQQLAQRQEAPKGEGLLSRLGAALARPFVAIIEWLGKLLGSRAHAATQAPLSRQDAPPAASLSAAEIKQMMLQKALPLTLGGLGKASELATLTAERLAKDHTRLASGDGALRSLATALVGIRDGSLIEASRTQAARLLEQSVGGIALQQWGTAGGAASQHVLSASPEQLREIAVQLHAVMDKVALLRHAVESEVKGEPVDKALADGLVEHFGLEAEQYLGEHPDGPYSDAEVMALGLYTNGEYQHLNRSLRQGRELDAGQALIDRGMSAAFEKSGPAEQVVKTFRGTQGRDAFEAVKEGQVGHDAGYLSTSRDPSVARSFAGLGTITTLFGRSGIDVSEISIEGDEQEILYDKGTDMRVLLSAKDGQGVTRRVLEEATLGERSGHSEGLLDALDLATGTDRSGKPQEQDLRLRMRGLDLA

SEQ ID NO: 29 - protein, 265 aa, unidentified
  REGION 1..265: note = Description of Unknown: CdtB toxin sequence
MKKIICLFLSFNLAFANLENFNVGTWNLQGSSAATESKWSVSVRQLVSGANPLDILMIQEAGTLPRTATPTGRHVQQGGTPIDEYEWNLGTLSRPDRVFIYYSRVDVGANRVNLAIVSRMQAEEVIVLPPPTTVSRPIIGIRNGNDAFFNIHALANGGTDVGAIITAVDAHFANMPQVNWMIAGDFNRDPSTITSTVDRELANRIRVVFPTSATQASGGTLDYAITGNSNRQQTYTPPLLAAILMLASLRSHIVSDHFPVNFRKF

SEQ ID NO: 30 - protein, 560 aa, Corynebacterium diphtheriae
MSRKLFASILIGALLGIGAPPSAHAGADDVVDSSKSFVMENFSSYHGTKPGYVDSIQKGIQKPKSGTQGNYDDDWKGFYSTDNKYDAAGYSVDNENPLSGKAGGVVKVTYPGLTKVLALKVDNAETIKKELGLSLTEPLMEQVGTEEFIKRFGDGASRVVLSLPFAEGSSSVEYINNWEQAKALSVELEINFETRGKRGQDAMYEYMAQACAGNRVRRSVGSSLSCINLDWDVIRDKTKTKIESLKEHGPIKNKMSESPNKTVSEEKAKQYLEEFHQTALEHPELSELKTVTGTNPVFAGANYAAWAVNVAQVIDSETADNLEKTTAALSILPGIGSVMGIADGAVHHNTEEIVAQSIALSSLMVAQAIPLVGELVDIGFAAYNFVESIINLFQVVHNSYNRPAYSPGHKTQPFLHDGYAVSWNTVEDSIIRTGFQGESGHDIKITAENTPLPIAGVLLPTIPGKLDVNKSKTHISVNGRKIRMRCRAIDGDVTFCRPKSPVYVGNGVHANLHVAFHRSSSEKIHSNEISSDSIGVLGYQKTVDHTKVNSKLSLFFEIKS

SEQ ID NO: 31 - protein, 621 aa, unidentified
  REGION 1..621: note = Description of Unknown: ExoU/VipB sequence
MKLAEIMTKSRKLKRNLLEISKTEAGQYSVSAPEHKGLVLSGGGAKGISYLGMIQALQERGKIKNLTHVSGASAGAMTASILAVGMDIKDIKKLIEGLDITKLLDNSGVGFRARGDRFRNILDVIYMMQMKKHLESVQQPIPPEQQMNYGILKQKIALYEDKLSRAGIVINNVDDIINLTKSVKDLEKLDKALNSIPTELKGAKGEQLENPRLTLGDLGRLRELLPEENKHLIKNLSVVVTNQTKHELERYSEDTTPQQSIAQVVQWSGAHPVLFVPGRNAKGEYIADGGILDNMPEIEGLDREEVLCVKAEAGTAFEDRVNKAKQSAMEAISWFKARMDSLVEATIGGKWLHATSSVLNREKVYYNIDNMIYINTGEVTTTNTSPTPEQRARAVKNGYDQTMQLLDSHKQTFDHPLMAILYIGHDKLKDALIDEKSEKEIFEASAHAQAILHLQEQIVKEMNDGDYSSVQNYLDQIEDILTVDAKMDDIQKEKAFALCIKQVNFLSEGKLETYLNKVEAEAKAAAEPSWATKILNLLWAPIEWVVSLFKGPAQDFKVEVQPEPVKVSTSENQETVSNQKDINPAVEYRKIIAEVRREHTDPSPSLQEKERVGLSTTFGGH

SEQ ID NO: 32 - protein, 211 aa, unidentified
  REGION 1..211: note = Description of Unknown: HopPtoE sequence
MNRVSGSSSATWQAVNDLVEQVSERTTLSTTGYQTAMGRLNKPEKSDADALMTMRRAQQYTDSAKRTYISETLMNLADLQQRKIYRTNSGNLRGAIEMTPTQLTDCVQKCREEGFSNCDIQALEIGLHLRHKLGISDFTIYSNRKLSHNYVVIHPSNAFPKGAIVDSWTGQGVVELDFKTRLKFKHREENYAVNANMHEWIERYGQAHVID

SEQ ID NO: 33 - protein, 204 aa, unidentified
  REGION 1..204: note = Description of Unknown: HopPtoF sequence
MGNICGTSGSRHVYSPSHTQRITSAPSTSTHVGGDTLTSIHQLSHSQREQFLNMHDPMRVMGLDHDTELFRTTDSRYIKNDKLAGNPQSMASILMHEELRPNRFASHTGAQPHEARAYVPKRIKATDLGVPSLNVMTGSLARDGIRAYDHMSDNQVSVKMRLGDFLERGGKVYADASSVADDGETSQALIVTLPKGQKVPVERV

SEQ ID NO: 34 - protein, 493 aa, unidentified
  REGION 1..493: note = Description of Unknown: HopPtoG sequence
MQIKNSHLYSASRMVQNTFNASPKMEVTNAIAKNNEPAALSATQTAKTHEGDSKGQSSNNSKLPFRAMRYAAYLAGSAYLYDKTANNFFLSTTSLHDGKGGFTSDARLNDAQDKARKRYQNNHSSTLENKNSLLSPLRLCGENQFLTMIDYRAATKIYLSDLVDTEQAHTSILKNIMCLKGELTNEEAIKKLNPEKTPKDYDLTNSEAYISKNKYSLTGVKNEETGSTGYTSRSITKPFVEKGLKHFIKATHGEKALTPKQCMETLDNLLRKSITLNSDSQFAAGQALLVFRQVYAGEDAWGDAERVILKSHYNRGTVLQDEADKIELSRPFSEQDLAKNMFKRNTSIAGPVLYHAYIYIQEKIFKLPPDKIEDLKHKSMADLKNLPLTHVKLSNSGVGFEDASGLGDSFTALNATSCVNHARIMSGEPPLSKDDVVILIGCLNAVYDNSSGIRHSLREIARGCFVGAGFTVQDGDDFYKQICKNASKQFYNG

SEQ ID NO: 35 - protein, 530 aa, Vibrio cholerae
MFKISVSQQANVMSTSDTAQRSSLKISIKSICNKSLSKKLHTLAEKCRRFSQELKEHTASKKQIVEQATTTVRESSLTKSDSELGSSRSLLTSDVLSSSSSHEDLTAVNLEDNDSVFVTIESSSELIVKQDGSIPPAPPLPGNIPPAPPLPSAGNIPTAPGLPKQKATTESVAQTSDNRSKLMEEIRQGVKLRATPKSSSTEKSASDPHSKLMKELINHGAKLKKVSTSDIPVPPPLPAAFASKPTDGRSALLSEIAGFSKDRLRKAGSSETLNVSQPTVAESSIPEAYDLLLSDEMFNLSPKLSETELNTLADSLADYLFKAADIDWMQVIAEQTKGSTQATSLKSQLEQAPEYVKAFCDEILKFPDCYKSADVASPESPKAGPSSVIDVALKRLQAGRNRLFSTIDAKGTNELKKGEAILESAINAARSVMTAEQKSALLSSNVKSATFKVFSELPCMEGFAEQNGKAAFNALRLAFYSSIQSGDTAQQDIARFMKENLATGFSGYSYLGLTSRVAQLEAQLAALTTK

SEQ ID NO: 36 - protein, 288 aa, Yersinia pestis
MIGPISQINISGGLSEKETSSLISNEELKNIITQLETDISDGSWFHKNYSRMDVEVMPALVIQANNKYPEMNLNLVTSPLDLSIEIKNVIENGVRSSRFIINMGEGGIHFSVIDYKHINGKTSLILFEPANFNSMGPAMLAIRTKTAIERYQLPDCHFSMVEMDIQRSSSECGIFSFALAKKLYIERDSLLKIHEDNIKGILSDGENPLPHDKLDPYLPVTFYKHTQGKKRLNEYLNTNPQGVGTVVNKKNETIVNRFDNNKSIVDGKELSVSVHKKRIAEYKTLLKV

SEQ ID NO: 37 - protein, 579 aa, unidentified
  REGION 1..579: note = Description of Unknown: AvrPtoB sequence
MAGINGAGPSGAYFVGHTDPEPASGGAHGSSSGASSSNSPRLPAPPDAPASQARDRREMLLRARPLSRQTREWVAQGMPPTAEAGVPIRPQESAEAAAPQARAEERHTPEADAAASHVRTEGGRTPQALAGTSPRHTGAVPHANRIVQQLVDAGADLAGINTMIDNAMRRHAIALPSRTVQSILIEHFPHLLAGELISGSELATAFRAALRREVRQQEASAPPRTAARSSVRTPERSTVPPTSTESSSGSNQRTLLGRFAGLMTPNQRRPSSASNASASQRPVDRSPPRVNQVPTGANRVVMRNHGNNEADAALQGLAQQGVDMEDLRAALERHILHRRPIPMDIAYALQGVGIAPSIDTGESLMENPLMNLSVALHRALGPRPARAQAPRPAVPVAPATVSRRPDSARATRLQVIPAREDYENNVAYGVRLLSLNPGAGVRETVAAFVNNRYERQAVVADIRAALNLSKQFNKLRTVSKADAASNKPGFKDLADHPDDATQCLFGEELSLTSSVQQVIGLAGKATDMSESYSREANKDLVFMDMKKLAQFLAGKPEHPMTRETLNAENIAKYAFRIVP

SEQ ID NO: 38 - protein, 1116 aa, unidentified
  REGION 1..1116: note = Description of Unknown: SdbA sequence
MHKKYNYYSLEKEKKTFWQHILDILKAPFRLPGWVVSFFLARNITHVALNPNNIPQQRLIHLTKTSNRPEDDIVVINFKKRPPHKWFNDTLIKIANTIAALPFVTPRLRTRLHYDNENDINHVNKLLAEIDALVQGKSKQKYCKGRAFDWSKIHLKGLEFLDPKMRGYVYEQLHEKYGYVSYTTKRKPNIEFFTLKTPDGSELDSVQVTGEDEEKKPMGERKFIITCIARDQNFINWIKDLNYTAKNLGATAISFNYRGVDYSRGLVWTENNLVDDILAQVQRLISLGADPKNICLDGMCIGGAVATIAAAKLHEKGMKVKLNNERSFTSLSSLVFGFIVPELQTANWWSPLTYGRFLLAGVVYALLTPLIWLAGWPVDVTKAWNRIPAQDKMYSVVRDKDNGLYDGVIHDHFCSIASLVDSQINSILYKLSTDQPLTEEEKQILCDDQFSHHFKPSQSVLKNPKYKGPHFISRQDLVAELGHREEYTNHDYFLDRLREKFQLDRATRPVALAEDGEKDIDGISSQLSNNKERPLIIASSGGTGHISATHGIINDLQSKTDNVVITQHHAELYKNKPFSITSVLIRIGVWFTSLPILEDILKGVMRFIGYPVLPSSSIFWDQMSKIQQSETKKENGIETGRTRPYVDMLLDIYPEGYEYTAFNNATHLTSSIEDIQTMISFKGHVEEDNRNIVYQNILQRLMHAAKQNTPYTRLISTQALSLGAICDAVKYYNTVFLPVYNAERGTSYQPIAIDQYMTDLPSLGCIHFMNNLEELTSEQRQLMEIHAVNMSEPFKEAHFGKEQGFKAVHNIDPRNNPMIRNAFKDPSLTKYLDKTQSFDLHFNVYKKEKQNALPVLNGKEKITIKPHAKIASIMIGSLAANASADYAKYLLNQGYEHIFLFGGLNDSIAARIDQIINSYPAPTRDEIRKKIILLGNQSDVEMAPIMTRSNCVVIRGGGLSVMEQMAMPIMDDKIVLLHHEDNEEGPLTSGLSWEDGNSDKLIEYLSEKGAYAKKTSPGLCSGHLHEAEKSFEKKYHGQLKSTETKKKVDLTIPQQETYSLKKEWDRKTGYTESGHILSHQHRFFNTIPEVREPFCSKEDLHHNELSSQSLVSVSAG

SEQ ID NO: 39 - protein, 965 aa, unidentified
  REGION 1..965: note = Description of Unknown: SidG sequence
MSRSKDEVLEANDSLFGITVQTWGTNDRPSNGMMNFADQQFFGGDVGHASINMKLPVTDKTKQWIEKYCYSQTYDQFKKVKGNEDKTYEEYLKTAKRLIPVELKTQVTRKAQYDSNGNLVTTHEKAYEQIYFDIDWSWWPGRLQNTEDDMVWEREGKHFEYDEKWKEYLQPEQRVHRGKLGSRKMDYAPTSIIHQRDIPTSELEKITRDHKIHTIEEKLNVVKLLQSKIDEMPHTKMSPSMELMFKNLGINVEKLLDETKDNGVDPTNLEAMREYLTNRLTERKLELETELSEAKKEVDSTQVKNKVEDVYYDFEYKLNQVRKKMEEVNSQLEKMDSLLHKLEGNTSGPIPYTAEIDELMSVLPFLKEELELENGTLSPKSIENLIDHIDELKNELASKQEKKNERNLNLIKKYEELCEQYKDDEEGLEEALWEEGIDVEEVNSAKKDISKPAPEIQKLTDLQEQLRNHKESGVKLSSELEETLNSSVKMWKTKIDSPCQVISESSVKALVSKINSTRPELVKEKEQLPEQEESLSKEAKKAQEELIKIQEFSQFYSENSSAYMVIGLPPHHQVSLPLAVNGKRGLHPEAMLKKMHELVAGPEKKEFNLHTNNCSLTSIEVLSAGAQHDPLLHSIMGTRALGFFGTPQQVLENAKLTSKTINEGKKSNIFTPLVTASPLDRALGYAMSIYMDPEASKAKQNAGLALGVLVGLAKTPGIIIGSLLNPKQGFNDILNTLNLVYSRNSTGLKVGLTLMALPAMIVLAPLAAIQKGVEVIAETIAKPFKLIANLFKQKPESTDEITVSVGSKKVAEKEGSYSNTALAGLVNSKIKSKIDENTITVEFQKSPQKMIEEFESQLKENPGKVVVLSEKAHNAVLKFVSKSDDEALKQKFYDCCNQSVARSQKFAPKTRDEIDELVEEVTSTDKTELTTSPRQEPSMSSTIDEEENIDSEHQIETGTESTMRI

SEQ ID NO: 40 - protein, 665 aa, unidentified
  REGION 1..665: note = Description of Unknown: VpdA sequence
MKTKQEVSQQDKLKDSKSSTPLQTKETWFISDALNITFDPYDFSISVTEQAPMPYRIVFSGGGSRILAHIGALDELTRHGLKFTEFSGSSAGAMVAAFAYLGYNCSEIKQIISWFNEDKLLDSPLIFNFNNIKQIFNKGGLSSAKLMRQAANYVILKKVMDIISDEKFKTRFAKFQNFLEENIYRCPENITFQTLARIKEICPECELGEKLFITGTNLSTQKHEVFSIDTTPSMALADAIIISANLPIAFERICYQGNVYSDGGISNNLPAHCFSEKGHKTTFLKHKDDVDFSVLALQFDNGLEENALYSQNPIPKWSWLSNTFYSLITGHPNVTENWYEDLQILRRHAHQSILIKTPTIALTNLTISQDTKKALVESGRTAAKTYLELHEFYTDDYGNIRHNECLHEKFQKPEELLDYCVLHSHFELLKKIKQAISCSQYLEKGYKHYLCELCDNLLPPQLKCPNEGSGTEQPEIKLEKDTIICEKNNNSGLTFSMTFFGVPSPLVKTLNQDSPELKIKLFTGLYPILIQNWQNLCPVSGISGILNSIRMSFVEISSTDTCIKTLIDKLNEIEIGHFLIFVFKAALKNYDKHDFILLLKNLKHLHHSIELIRNKPFHSDDRFYGQWSFEGHDPKRILEFIKSDDISGLMTILEDKKALPNNKPN

SEQ ID NO: 41 - protein, 246 aa, Legionella pneumophila
MVSLEHIQKLISECRKLGKDGLDNGTNGLIPELEIDVVPPSAFLGVGNNPAIFVNSKTYKLMRTTHEKWVENKTIVFKSYLLSQPAIKIIGAIVHETGHAFNVAAKIPNTEANACIFEIEVLMRLFQVKSPLLLGCTELDMQSYFKSRLTDYNKCVKDCQCLAEMVEFITHQFKLDEVSISEKENQIPLLSISNKWPGLFAKKQIAPDMDKLLTSPVTITPEVKILFYQLVKEHFHSPETEIKLDI

SEQ ID NO: 42 - protein, 644 aa, Legionella pneumophila
MYKIYSYLGWRIDMKTENLPQAGQEAQIDKKIHFIWVGHIMPQKNIQVVSEWAEKNPGYETIIWVDKKIAPAKELDLFILDMKSKGITVKDINEEGVCRDSIRHELDQESPNYGMVSDMLRLNILAAEGGIYLDSDILCSAPFPDEIYAPFGFLLSPWSQGANNTLCNDIILCSKGNQIIQQLADAIEQSYIARDSFEFTHEYASMKETKGERIAKTLGVTGPGFLFHQLKKMGILNDKSEMEAIHWELQDQRYLIDGSVKEPDYFYVPQNNTNDASWVPSIKRPGIENMSFQERLENAVQLIAFDIQKTGLFNLDHYANELKVKQNSWCIAAETSPELKPDSYLLIRPRDKTGEWTLYYVDEDKKLNPVTLPVIKGAIKLSEVSDPLRKFHTLLSQVSDPVNPTAHELKQIGRALIELKPRQDEWHCKNKWSGAEEIAQELWQRITSNETLRAQIKQCFTQFESLKPRVAELGLTRASGAGTEVEAHESTVKEQEIISQNTVGEEGTKEKNSVQLASENSSDEKIKTAHDLIDEIIQDVIQLDGKLGLLGGNTRQLEDGRVINIPNGAAMIFDDYKKYKQGELTAESALESMIKIAKLSNQLNRHTFFNQRQPETGQFYKKVAAIDLQTTIAAEYDNNHGLRI

SEQ ID NO: 43 - protein, 219 aa, Yersinia enterocolitica
MKISSFISTSLPLPTSVSGSSSVGEMSGRSVSQQTSDQYANNLAGRTESPQGSSLASRIIERLSSVAHSVIGFIQRMFSEGSHKPVVTPAPTPAQMPSPTSFSDSIKQLAAETLPKYMQQLNSLDAEMLQKNHDQFATGSGPLRGSITQCQGLMQFCGGELQAEASAILNTPVCGIPFSQWGTIGGAASAYVASGVDLTQAANEIKGLAQQMQKLLSLM

SEQ ID NO: 44 - protein, 543 aa, Salmonella typhimurium
MLKYEERKLNNLTLSSFSKVGVSNDARLYIAKENTDKAYVAPEKFSSKVLTWLGKMPLFKNTEVVQKHTENIRVQDQKILQTFLHALTEKYGETAVNDALLMSRINMNKPLTQRLAVQITECVKAADEGFINLIKSKDNVGVRNAALVIKGGDTKVAEKNNDVGAESKQPLLDIALKGLKRTLPQLEQMDGNSLRENFQEMASGNGPLRSLMTNLQNLNKIPEAKQLNDYVTTLTNIQVGVARFSQWGTCGGEVERWVDKASTHELTQAVKKIHVIAKELKNVTAELEKIEAGAPMPQTMSGPTLGLARFAVSSIPINQQTQVKLSDGMPVPVNTLTFDGKPVALAGSYPKNTPDALEAHMKMLLEKECSCLVVLTSEDQMQAKQLPPYFRGSYTFGEVHTNSQKVSSASQGEAIDQYNMQLSCGEKRYTIPVLHVKNWPDHQPLPSTDQLEYLADRVKNSNQNGAPGRSSSDKHLPMIHCLGGVGRTGTMAAALVLKDNPHSNLEQVRADFRDSRNNRMLEDASQFVQLKAMQAQLLMTTAS

SEQ ID NO: 45 - protein, 240 aa, Salmonella typhimurium
MTNITLSTQHYRIHRSDVEPVKEKTTEKDIFAKSITAVRNSFISLSTSLSDRFSLHQQTDIPTTHFHRGNASEGRAVLTSKTVKDFMLQKLNSLDIKGNASKDPAYARQTCEAILSAVYSNNKDQCCKLLISKGVSITPFLKEIGEAAQNAGLPGEIKNGVFTPGGAGANPFVVPLIASASIKYPHMFINHNQQVSFKAYAEKIVMKEVTPLFNKGTMPTPQQFQLTIENIANKYLQNAS

SEQ ID NO: 46 - protein, 561 aa, Salmonella typhimurium
MQIQSFYHSASLKTQEAFKSLQKTLYNGMQILSGQGKAPAKAPDARPEIIVLREPGATWGNYLQHQKASNHSLHNLYNLQRDLLTVAATVLGKQDPVLTSMANQMELAKVKADRPATKQEEAAAKALKKNLIELIAARTQQQDGLPAKEAHRFAAVAFRDAQVKQLNNQPWQTIKNTLTHNGHHYTNTQLPAAEMKIGAKDIFPSAYEGKGVCSWDTKNIHHANNLWMSTVSVHEDGKDKTLFCGIRHGVLSPYHEKDPLLRHVGAENKAKEVLTAALFSKPELLNKALAGEAVSLKLVSVGLLTASNIFGKEGTMVEDQMRAWQSLTQPGKMIHLKIRNKDGDLQTVKIKPDVAAFNVGVNELALKLGFGLKASDSYNAEALHQLLGNDLRPEARPGGWVGEWLAQYPDNYEVVNTLARQIKDIWKNNQHHKDGGEPYKLAQRLAMLAHEIDAVPAWNCKSGKDRTGMMDSEIKREIISLHQTHMLSAPGSLPDSGGQKIFQKVLLNSGNLEIQKQNTGGAGNKVMKNLSPEVLNLSYQKRVGDENIWQSVKGISSLITS

SEQ ID NO: 47 - protein, 685 aa, Salmonella typhimurium
MVTSVRTQPPVIMPGMQTEIKTQATNLAANLSAVRESATTTLSGEIKGPQLEDFPALIKQASLDALFKCGKDAEALKEVFTNSNNVAGKKAIMEFAGLFRSALNATSDSPEAKTLLMKVGAEYTAQIIKDGLKEKSAFGPWLPETKKAEAKLENLEKQLLDIIKNNTGGELSKLSTNLVMQEVMPYIASCIEHNFGCTLDPLTRSNLTHLVDKAAAKAVEALDMCHQKLTQEQGTSVGREARHLEMQTLIPLLLRNVFAQIPADKLPDPKIPEPAAGPVPDGGKKAEPTGINININIDSSNHSVDNSKHINNSRSHVDNSQRHIDNSNHDNSRKTIDNSRTFIDNSQRNGESHHSTNSSNVSHSHSRVDSTTHQTETAHSASTGAIDHGIAGKIDVTAHATAEAVTNASSESKDGKVVTSEKGTTGETTSFDEVDGVTSKSIIGKPVQATVHGVDDNKQQSQTAEIVNVKPLASQLAGVENVKTDTLQSDTTVITGNKAGTTDNDNSQTDKTGPFSGLKFKQNSFLSTVPSVTNMHSMHFDARETFLGVIRKALEPDTSTPFPVRRAFDGLRAEILPNDTIKSAALKAQCSDIDKHPELKAKMETLKEVITHHPQKEKLAEIALQFAREAGLTRLKGETDYVLSNVLDGLIGDGSWRAGPAYESYLNKPGVDRVITTVDGLHMQR

SEQ ID NO: 48 - protein, 732 aa, Yersinia pestis
MKSVKIMGTMPPSISLAKAHERISQHWQNPVGELNIGGKRYRIIDNQVLRLNPHSGFSLFREGVGKIFSGKMFNFSIARNLTDTLHAAQKTTSQELRSDIPNALSNLFGAKPQTELPLGWKGEPLSGAPDLEGMRVAETDKFAEGESHISIIETKDKQRLVAKIERSIAEGHLFAELEAYKHIYKTAGKHPNLANVHGMAVVPYGNRKEEALLMDEVDGWRCSDTLRTLADSWKQGKINSEAYWGTIKFIAHRLLDVTNHLAKAGVVHNDIKPGNVVFDRASGEPVVIDLGLHSRSGEQPKGFTESFKAPELGVGNLGASEKSDVFLVVSTLLHCIEGFEKNPEIKPNQGLRFITSEPAHVMDENGYPIHRPGIAGVETAYTRFITDILGVSADSRPDSNEARLHEFLSDGTIDEESAKQILKDTLTGEMSPLSTDVRRITPKKLRELSDLLRTHLSSAATKQLDMGGVLSDLDTMLVALDKAEREGGVDKDQLKSFNSLILKTYRVIEDYVKGREGDTKNSSTEVSPYHRSNFMLSIVEPSLQRIQKHLDQTHSFSDIGSLVRAHKHLETLLEVLVTLSQQGQPVSSETYGFLNRLAEAKITLSQQLNTLQQQQESAKAQLSILINRSGSWADVARQSLQRFDSTRPVVKFGTEQYTAIHRQMMAAHAAITLQEVSEFTDDMRNFTVDSIPLLIQLGRSSLMDEHLVEQREKLRELTTIAERLNRLEREWM

SEQ ID NO: 49 - protein, 529 aa, Yersinia pestis
MFINPRNVSNTFLQEPLRHSSNLTEMPVEAENVKSKTEYYNAWSEWERNAPPGNGEQREMAVSRLRDCLDRQAHELELNNLGLSSLPELPPHLESLVASCNSLTELPELPQSLKSLQVENNNLKALPDLPPSLKKLHVRENDLTDLPELPQSLESLRVDNNNLKALSDLPPSLEYLTASSNKLEELPELQNLPFLAAIYADNNLLETLPDLPPSLKKLHVRENDLTDLPELPQSLESLQVDNNNLKALSDLPPSLEYLTASSNKLEELPELQNLPFLAAIYADNNLLETLPDLPPHLEILVASYNSLTELPELPQSLKSLRVDNNNLKALSDLPPSLEYLTASSNKLEELPELQNLPFLAAIYADNNLLETLPDLPPSLKKLHVRENDLTDLPELPQSLTFLDVSDNNISGLSELPPNLYYLDASSNEIRSLCDLPPSLVDLNVKSNQLSELPALPPHLERLIASFNYLAEVPELPQNLKQLHVEQNALREFPDIPESLEELEMDSERVVDPYEFAHETTDKLEDDVFE

SEQ ID NO: 50 - protein, 35 aa, unidentified
  REGION 1..35: note = Description of Unknown: Amatoxin sequence
MSDINATRLPIWGIGCNPCVGDDVTTLLTRGEALC

SEQ ID NO: 51 - protein, 34 aa, Amanita fuliginea
MSDINATRLPAWLVDCPCVGDDVNRLLTRGESLC

SEQ ID NO: 52 - protein, 291 aa, Ustilago maydis
MIKPERSILTILIGILCLLAYVLANGEPHDGDNEWSSYCSDQGFRRSDDGLVTTPDVGQESIGKNSINGSELVDYLQCLKVRLNGQKQVVSNDGWLLLLVQEPSVNVTQKAMSECNYNVSSGHKAGSYIQVTNTPADYKVISRRGSYEGDQLPEDVKPYFGVQKTSDYRPISKRINPNLTLRQLAYNFAALNMCSLWCNSCISRSCPYYIAELTVHVNNIHHGTVWLHHFCRNASPQGGNLYSTLTISHKDTAYYVGTGWWKVRSTAATTNDVAGDWYPASWNQYWCGPHY

SEQ ID NO: 53 - protein, 219 aa, Ustilago maydis
MLIFSVLMYLGLLLAGASALPNGLSPRNNAFCAGFGLSCKWECWCTAHGTGNELRYATAAGCGDHLSKSYYDARAGHCLFSDDLRNQFYSHCSSLNNNMSCRSLSKRTIQDSATDTVDLGAELHRDDPPPTASDIGKRGKRPRPVMCQCVDTTNGGVRLDAVTRAACSIDSFIDGYYTEKDGFCRAKYSWDLFTSGQFYQACLRYSHAGTNCQPDPQYE

SEQ ID NO: 54 - protein, 316 aa, Saccharomyces cerevisiae
MTKPTQVLVRSVSILFFITLLHLVVALNDVAGPAETAPVSLLPREAPWYDKIWEVKDWLLQRATDGNWGKSITWGSFVASDAGVVIFGINVCKNCVGERKDDISTDCGKQTLALLVSIFVAVTSGHHLIWGGNRPVSQSDPNGATVARRDISTVADGDIPLDFSALNDILNEHGISILPANASQYVKRSDTAEHTTSFVVTNNYTSLHTDLIHHGNGTYTTFTTPHIPAVAKRYVYPMCEHGIKASYCMALNDAMVSANGNLYGLAEKLFSEDEGQWETNYYKLYWSTGQWIMSMKFIEESIDNANNDFEGCDTGH

SEQ ID NO: 55 - protein, 296 aa, Saccharomyces cerevisiae
MGHLAILFSIIAVLNIATAVASSDSIYLKGHRVGQDIDSLYRVYDNGTMYPVTFNEWLNDLTGMNDLATNNATILKRDSSDVSCVTETCQYVDYHVDDEGVITIDISTYRIPVEWDSGSAGNASYGVSKRDTKYETFCKKKICGINVSGFCNAYDFAVHAFDFGGSVYNPVSGITDRIKEATKRDKTECLGYELDHVRIDPAVDWSISISTWKQGSANCDTQASADSLKCAAQKALESEHNHQKTAFCIHLDNGGSFNLDIRLISELSFSKYNPWALPCPKYKGSNSWQVVSDCFQ

SEQ ID NO: 56 - protein, 708 aa, Saccharomyces cerevisiae
MPRFAIIFALLIAYSLFLSTLFTGSIPDRANTVTSNAPCQVVIWDWIRTRRICNCCSRLCYSLLGRSNLSRTAKRGVCTIAGAVLATAAVIVAAVLVGKSSGSATKRGLTKTISVLNHTIPFTDHILNGQTLSNGTGSNFVTIGFSGYAVHATIKRASTTDIISWVIPESMEPTLARVASYVSSSSINLAAVPDTGGNASALSFQNAVQEFATSWVSMTYDQSYGDLRNVANDEGGEEILILMRKRSYRISFQVIETGSTALLLRTRRVVSQLITMTYLVTVQARVGIQIGDIFQHYGGIDNYVMTSISVLRTLEDKAFHENKLLIVREPPNKSNQDANQSYRLRPFSANDLIQNLKSVDIGFLAFCSFFDKYAHYPEIIMMKITIFISKGNLWSIIYVIQARYVRKRVMKVRGQMPGGLLTNMESLLNIVSTPNLNISEFHIQTHSMSQSKPMYFQKQCYSSQNNIIYIYNSIHITCGAVYVIVHDVRTPSVFVLIELRNCKPLKNSWCETTKTSPRDTKIKKNEYNETVCRRAGALLDGRVRTIRFLMMRTHWSRVKGVSCNTANRLSRFCNHVVSYYPSQNATIHLLPTSLRAESLEQQYTTRPLSSSNNRFCCLKSIFINNCKKACESPSLVSCNLQQTAELLMVYYLYICEACYVSRNHDLLSKQCMSTVRAVYVARMRLPKFRSTFPCMPRLCWLVNGVVVV

SEQ ID NO: 57 - protein, 768 aa, Bacillus anthracis
MHVKEKEKNKDENKRKDEERNKTQEEHLKEIMKHIVKIEVKGEEAVKKEAAEKLLEKVPSDVLEMYKAIGGKIYIVDGDITKHISLEALSEDKKKIKDIYGKDALLHEHYVYAKEGYEPVLVIQSSEDYVENTEKALNVYYEIGKILSRDILSKINQPYQKFLDVLNTIKNASDSDGQDLLFTNQLKEHPTDFSVEFLEQNSNEVQEVFAKAFAYYIEPQHRDVLQLYAPEAFNYMDKFNEQEINLSLEELKDQRMLSRYEKWEKIKQHYQHWSDSLSEEGRGLLKKLQIPIEPKKDDIIHSLSQEEKELLKRIQIDSSDFLSTEEKEFLKKLQIDIRDSLSEEEKELLNRIQVDSSNPLSEKEKEFLKKLKLDIQPYDINQRLQDTGGLIDSPSINLDVRKQYKRDIQNIDALLHQSIGSTLYNKIYLYENMNINNLTATLGADLVDSTDNTKINRGIFNEFKKNFKYSISSNYMIVDINERPALDNERLKWRIQLSPDTRAGYLENGKLILQRNIGLEIKDVQIIKQSEKEYIRIDAKVVPKSKIDTKIQEAQLNINQEWNKALGLPKYTKLITFNVHNRYASNIVESAYLILNEWKNNIQSDLIKKVTNYLVDGNGRFVFTDITLPNIAEQYTHQDEIYEQVHSKGLYVPESRSILLHGPSKGVELRNDSEGFIHEFGHAVDDYAGYLLDKNQSDLVTNSKKFIDIFKEEGSNLTSYGRTNEAEFFAEAFRLMHSTDHAERLKVQKNAPKTFQFINDQIKFIINS

SEQ ID NO: 58 - protein, 319 aa, unidentified
  REGION 1..319: note = Description of Unknown: Shiga Toxin sequence
MKCILLKWVLCLLLGFSSVSYSREFTIDFSTQQSYVSSLNSIRTEISTPLEHISQGTTSVSVINHTPPGSYFAVDIRGLDVYQARFDHLRLIIEQNNLYVAGFVNTATNTFYRFSDFAHISVPGVTTVSMTTDSSYTTLQRVAALERSGMQISRHSLVSSYLALMEFSGNTMTRDASRAVLRFVTVTAEALRFRQIQREFRQALSETAPVYTMTPGDVDLTLNWGRISNVLPEYRGEDGVRVGRISFNNISAILGTVAVILNCHHQGARSVRAVNEESQPECQITGDRPVIKINNTLWESNTAAAFLNRKSQSLYTTGE

SEQ ID NO: 59 - protein, 565 aa, Ricinus communis
MYAVATWLCFGSTSGWSFTLEDNNIFPKQYPIINFTTAGATVQSYTNFIRAVRGRLTTGADVRHDIPVLPNRVGLPINQRFILVELSNHAELSVTLALDVTNAYVVGYRAGNSAYFFHPDNQEDAEAITHLFTDVQNRYTFAFGGNYDRLEQLAGNLRENIELGNGPLEEAISALYYYSTGGTQLPTLARSFIICIQMISEAARFQYIEGEMRTRIRYNRRSAPDPSVITLENSWGRLSTAIQESNQGAFASPIQLQRRNGSKFSVYDVSILIPIIALMVYRCAPPPSSQFSLLIRPVVPNFNADVCMDPEPIVRIVGRNGLCVDVRDGRFHNGNAIQLWPCKSNTDANQLWTLKRDNTIRSNGKCLTTYGYSPGVYVMIYDCNTAATDATRWQIWDNGTIINPRSSLVLAATSGNSGTTLTVQTNIYAVSQGWLPTNNTQPFVTTIVGLYGLCLQANSGQVWIEDCSSEKAEQQWALYADGSIRPQQNRDNCLTSDSNIRETVVKILSCGPASSGQRWMFKNDGTILNLYSGLVLDVRRSDPSLKQIILYPLHGDPNQIWLPLF

SEQ ID NO: 60 - DNA, 98 bp, synthetic construct
  source 1..98: mol_type = other DNA
  CDS 1..72
  misc_feature 1..98: note = Description of Artificial Sequence: Synthetic oligonucleotide
aagggtgacgctgaaagatgggtttctggtccaggcgcgccacttctaaataagcgaatttcttatgatttatgatttttattattaaataagttata

SEQ ID NO: 61 - DNA, 112 bp, synthetic construct
  source 1..112: mol_type = other DNA
  CDS 1..111
  misc_feature 1..112: note = Description of Artificial Sequence: Synthetic polynucleotide
gagcagaagctaatctcagaggaggacctgtttaaaccaggaggcggttctggtccaggtactgaagacgctgaagctgttgctttgggtttgggtttgtctgacttcccat

SEQ ID NO: 62 - DNA, 114 bp, synthetic construct
  modified_base 33..62: mod_base = OTHER; note = n = a, c, t, g, unknown or other
  source 1..114: mol_type = other DNA
  CDS 69..113
  misc_feature 1..114: note = Description of Artificial Sequence: Synthetic polynucleotide
aacgtcaaggagaaaaaactataatggttaatnnnnnnnnnnnnnnnnnnnnnnnnnnnnnntaatagacaagctacgttgaaacaagaacccgcctcctttcagaactcactt

SEQ ID NO: 63 - DNA, 7737 bp, synthetic construct
  source 1..7737: mol_type = other DNA
  misc_feature 1..7737: note = Description of Artificial Sequence: Synthetic polynucleotide
tcgcgcgtttcggtgatgacggtgaaaacctctgacacatgcagctcccggagacggtcacagcttgtctgtaagcggatgccgggagcagacaagcccgtcagggcgcgtcagcgggtgttggcgggtgtcggggctggcttaactatgcggcatcagagcagattgtactgagagtgcaccatatgcggtgtgaaataccgcacagatgcgtaaggagaaaataccgcatcaggcgccattcgccattcaggctgcgcaactgttgggaagggcgatcggtgcgggcctcttcgctattacgccagctggcgaaagggggatgtgctgcaaggcgattaagttgggtaacgccagggttttcccagtcacgacgttgtaaaacgacggccagtgaattcgagctcggtacccgtcttctgtcccagttaccgaatctaagggcactaccaccaaagaaacaggtgttactaccaaacaaaccacagccaacccaagtctaaccgtctccacagtcgtcccagtttcatcctctgcttcttctcattccgttgtcatcaacagtaacggtgctaacgtcgtcgttccaggtgctttaggtttggctggtgttgctatgttattcttataaacggtggtgtttgacacatccgccttcttaatgctttctttcagtattatgttatttttttgttattcgtttttcacttctaggctttttgacagactagccccgttataccaccatctttgtgggaaagcccctaaattgccctgagcagtatcgtttcatgtctagtctctttaaagatgtttcttacacttctcctatgcacatatattaattaaagtccaatgctagtagagaaggggggtaacacccctccgcgctcttttccgatttttttctaaaccgtggaatatttcggatatccttttgttgtttccgggtgtacaatatggacttcctcttttctggcaaccaaacccatacatcgggattcctataataccttcgttggtctccctaacatgtaggtggcggaggggagatatacaatagaacagataccagacaagacataatgggctaaacaagactacaccaattacactgcctcattgatggtggtacataacgaactaatactgtagccctagacttgatagccatcatcatatcgaagtttcactaccctttttccatttgccatctattgaagtaataataggcgcatgcaacttcttttctttttttttcttttctctctcccccgttgttgtctcaccatatccgcaatgacaaaaaaatgatggaagacactaaaggaaaaaattaacgacaaagacagcaccaacagatgtcgttgttccagagctgatgaggggtatctcgaagcacacgaaactttttccttccttcattcacgcacactactctctaatgagcaacggtatacggccttccttccagttacttgaatttgaaataaaaaaaagtttgctgtcttgctatcaagtataaatagacctgcaattattaatcttttgtttcctcgtcattgttctcgttccctttcttccttgtttctttttctgcacaatatttcaagctataccaagcatacaatcaactccaagctttgcaaagatggggtcaaaggccgagctaatcccagagccccctaaaaaaaagagaaaggtcgagctgggaactgcggcagagtacccgtatgatgtaccggactatgccggaggtatgtctagattggacaagtctaaggttatcaactctgctttggaattgttgaacgaagttggtatcgaaggtttgactactagaaagttggctcaaaagttgggtgttgaacaaccaactttgtactggcacgttaagaacaagagagctttgttggacgctttggctatcgaaatgttggacagacaccacactcacttctgtccattggaaggtgaatcttggcaagacttcttgagaaacaacgctaagtctttcagatgtgctttgttgtctcacagagacggtgctaaggttcacttgggtactagaccaactgaaaagcaatacgaaactttggaaaaccaattggctttcttgtgtcaacaaggtttctctttggaaaacgctttgtacgctttgtctgctgttggtcacttcactttgggttgtgttttggaagaccaagaacaccaagttgctaaggaagaaagagaaactccaactactgactctatgccaccattgttgagacaagctatcgaattgttcgaccaccaaggtgctgaaccagctttcttgttcggtttggaattgatcatctgtggtttggaaaagcaattgaagtgtgaatctggttctgggcaaccatctttgagatctgaatacgaatacccagttttctctcacgttcaagctggtatgttctctccagaattgagaactttcactaagggtgacgctgaaagatgggtttctggtccaggcgcgccacttctaaataagcgaatttcttatgatttatgatttttattattaaataagttataaaaaaaataagtgtatacaaattttaaagtgactcttaggttttaaaacgaaaattcttattcttgagtaactctttcctgtaggtcaggttgctttctcaggtatagcatgaggtcgctcttattgaccacacctctaccggcagatctgtacaatcttgatccggagcttttctttttttgccgattaagaattaattcggtcgaaaaaagaaaaggagagggccaagagggagggcattggtgactattgagcacgtgagtatacgtgattaagcacacaaaggcagcttggagtatgtctgttattaatttcacaggtagttctggtccattggtgaaagtttgcggcttgcagagcacagaggccgcagaatgtgctctagattccgatgctgacttgctgggtattatatgtgtgcccaatagaaagagaacaattgacccggttattgcaaggaaaatttcaagtcttgtaaaagcatataaaaatagttcaggcactccgaaatacttggttggcgtgtttcgtaatcaacctaaggaggatgttttggctctggtcaatgattacggcattgatatcgtccaactgcatggagatgagtcgtggcaagaataccaagagttcctcggtttgccagttattaaaagactcgtatttccaaaagactgcaacatactactcagtgcagcttcacagaaacctcattcgtttattcccttgtttgattcagaagcaggtgggacaggtgaacttttggattggaactcgatttctgactgggttggaaggcaagagagccccgaaagcttacattttatgttagctggtggactgacgccagaaaatgttggtgatgcgcttagattaaatggcgttattggtgttgatgtaagcggaggtgtggagacaaatggtgtaaaagactctaacaaaatagcaaatttcgtcaaaaatgctaagaaataggttattactgagtagtatttatttaagtattgtttgtgcacttgcctgcggtgtgaaataccgcacagatgcgtaaggaatatttcggatatccttttgttgtttccgggtgtacaatatggacttcctcttttctggcaaccaaacccatacatcgggattcctataataccttcgttggtctccctaacatgtaggtggcggaggggagatatacaatagaacagataccagacaagacataatgggctaaacaagactacaccaattacactgcctcattgatggtggtacataacgaactaatactgtagccctagacttgatagccatcatcatatcgaagtttcactaccctttttccatttgccatctattgaagtaataataggcgcatgcaacttcttttctttttttttcttttctctctcccccgttgttgtctcaccatatccgcaatgacaaaaaaatgatggaagacactaaaggaaaaaattaacgacaaagacagcaccaacagatgtcgttgttccagagctgatgaggggtatctcgaagcacacgaaactttttccttccttcattcacgcacactactctctaatgagcaacggtatacggccttccttccagttacttgaatttgaaataaaaaaaagtttgctgtcttgctatcaagtataaatagacctgcaattattaatcttttgtttcctcgtcattgttctcgttccctttcttccttgtttctttttctgcacaatatttcaagctataccaagcatacaatcaactccaagctttgcaaagatggggtcaaaggccgagctaatcccagagccccctaaaaaaaagagaaaggtcgagctgggaactgcggcagaggagcagaagctgatctcagaggaggacctgtttaaaccaggaggcggttctggtccaggtactgaagacgctgaagctgttgctttgggtttgggtttgtctgacttcccatctgctggtaaggctgttttggacgacgaagactctttcgtttggccagctgcttctttcgacatgggtgcttgttgggctggtgctggtttcgctgacccagacccagcttgtatcttcttgaacttgccatgagcccatcttttttttggacctaaattcttcatgaaaatatattacgagggcttattcagaagctttggacttcttcgccagaggtttggtcaagtctccaatcaaggttgtcggcttgtctaccttgccagaaatttacgaaaagatggaaaagggtcaaatcgttggtagatacgttgttgacacttctaaataagcgaatttcttatgatttatgatttttattattaaataagttataaaaaaaataagtgtatacaaattttaaagtgactcttaggttttaaaacgaaaattcttattcttgagtaactctttcctgtaggtcaggttgctttctcaggtatagcatgaggtcgctcttattgaccacacctctaccggccggtcgaaattcccctaccctatgaacatattccattttgtaatttcgtgtcgcgttgcgtgtaaaacatcctctcattcaagacagggttttctaaaagcaataggggtagtttaataattcttatataatcatcatatacactatttttagttcttaattctttaatacaaacttattaatgtgctctccattgatctcttaatcaggaggcgatatataccggaagcggtgtacttttcttcacctcttactcaactatgttgatgtgcaagtttaaccactcgtcgatattatctattgctataacgaaaactttattcgagttcacagtgaaaaacttcagcacatttatggaagatctaagcaaaatggagaacgccagtagatgcgaacaacaaactttatcaaatttgaaataccactgctttgataagctatagcttggcgtaatcatggtcatagctgtttcctgtgtgaaattgttatccgctcacaattccacacaacatacgagccggaagcataaagtgtaaagcctggggtgcctaatgagtgagctaactcacattaattgcgttgcgctcactgcccgctttccagtcgggaaacctgtcgtgccagctgcattaatgaatcggccaacgcgcggggagaggcggtttgcgtattgggcgctcttccgcttcctcgctcactgactcgctgcgctcggtcgttcggctgcggcgagcggtatcagctcactcaaaggcggtaatacggttatccacagaatcaggggataacgcaggaaagaacatgtgagcaaaaggccagcaaaaggccaggaaccgtaaaaaggccgcgttgctggcgtttttccataggctccgcccccctgacgagcatcacaaaaatcgacgctcaagtcagaggtggcgaaacccgacaggactataaagataccaggcgtttccccctggaagctccctcgtgcgctctcctgttccgaccctgccgcttaccggatacctgtccgcctttctcccttcgggaagcgtggcgctttctcatagctcacgctgtaggtatctcagttcggtgtaggtcgttcgctccaagctgggctgtgtgcacgaaccccccgttcagcccgaccgctgcgccttatccggtaactatcgtcttgagtccaacccggtaagacacgacttatcgccactggcagcagccactggtaacaggattagcagagcgaggtatgtaggcggtgctacagagttcttgaagtggtggcctaactacggctacactagaagaacagtatttggtatctgcgctctgctgaagccagttaccttcggaaaaagagttggtagctcttgatccggcaaacaaaccaccgctggtagcggtggtttttttgtttgcaagcagcagattacgcgcagaaaaaaaggatctcaagaagatcctttgatcttttctacggggtctgacgctcagtggaacgaaaactcacgttaagggattttggtcatgagattatcaaaaaggatcttcacctagatccttttaaattaaaaatgaagttttaaatcaatctaaagtatatatgagtaaacttggtctgacagttaccaatgcttaatcagtgaggcacctatctcagcgatctgtctatttcgttcatccatagttgcctgactccccgtcgtgtagataactacgatacgggagggcttaccatctggccccagtgctgcaatgataccgcgagacccacgctcaccggctccagatttatcagcaataaaccagccagccggaagggccgagcgcagaagtggtcctgcaactttatccgcctccatccagtctattaattgttgccgggaagctagagtaagtagttcgccagttaatagtttgcgcaacgttgttgccattgctacaggcatcgtggtgtcacgctcgtcgtttggtatggcttcattcagctccggttcccaacgatcaaggcgagttacatgatcccccatgttgtgcaaaaaagcggttagctccttcggtcctccgatcgttgtcagaagtaagttggccgcagtgttatcactcatggttatggcagcactgcataattctcttactgtcatgccatccgtaagatgcttttctgtgactggtgagtactcaaccaagtcattctgagaatagtgtatgcggcgaccgagttgctcttgcccggcgtcaatacgggataataccgcgccacatagcagaactttaaaagtgctcatcattggaaaacgttcttcggggcgaaaactctcaaggatcttaccgctgttgagatccagttcgatgtaacccactcgtgcacccaactgatcttcagcatcttttactttcaccagcgtttctgggtgagcaaaaacaggaaggcaaaatgccgcaaaaaagggaataagggcgacacggaaatgttgaatactcatactcttcctttttcaatattattgaagcatttatcagggttattgtctcatgagcggatacatatttgaatgtatttagaaaaataaacaaataggggttccgcgcacatttccccgaaaagtgccacctgacgtctaagaaaccattattatcatgacattaacctataaaaataggcgtatcacgaggccctttcgtc

SEQ ID NO: 64 - DNA, 10004 bp, synthetic construct
  modified_base 1458..2224: mod_base = OTHER; note = n = a, c, t, g, unknown or other
  modified_base 2945..2974: mod_base = OTHER; note = n = a, c, t, g, unknown or other
  source 1..10004: mol_type = other DNA
  misc_feature 1..10004: note = Description of Artificial Sequence: Synthetic polynucleotide
tgcatgcctgcaggtcgagatccgggatcgaagaaatgatggtaaatgaaataggaaatcaaggagcatgaaggcaaaagacaaatataagggtcgaacgaaaaataaagtgaaaagtgttgatatgatgtatttggctttgcggcgccgaaaaaacgagtttacgcaattgcacaatcatgctgactctgtggcggacccgcgctcttgccggcccggcgataacgctgggcgtgaggctgtgcccggcggagttttttgcgcctgcattttccaaggtttaccctgcgctaaggggcgagattggagaagcaataagaatgccggttggggttgcgatgatgacgaccacgacaactggtgtcattatttaagttgccgaaagaacctgagtgcatttgcaacatgagtatactagaagaatgagccaagacttgcgagacgcgagtttgccggtggtgcgaacaatagagcgaccatgaccttgaaggtgagacgcgcataaccgctagagtactttgaagaggaaacagcaatagggttgctaccagtataaatagacaggtacatacaacactggaaatggttgtctgtttgagtacgctttcaattcatttgggtgtgcactttattatgttacaatatggaagggaactttacacttctcctatgcacatatattaatcataagttgaattcgacaggttatcagcaacaacacagtcatatccattctcaattagctctaccacagtgtgtgaaccaatgtatccagcaccacctgtaaccaaaacaattttacctcgatcgagtttaccactccctatcagtgatagagaaaagttaaagtcgagtttaccactccctatcagtgatagagaacagtcaaagtcgagtttaccactccctatcagtgatagagaaaagttaaagtcgagtttaccactccctatcagtgatagagaaaagttaaagtcgagtttaccactccctatcagtgatagagaacagtcaaagtcgagtttaccactccctatcagtgatagagaattgtgaaagtcgagtttaccactccctatcagtgatagagaaaagtccaagtcgagctcggtaccctatggcatgcatgtggatgataatgcgattagttttttagccttatttctggggtaattaatcagcgaagcgatgatttttgatctattaacagatatataaatggaaaagctgcataaccactttaactaatactttcaacattttcagtttgtattacttcttattcaaatgtcataaaagtatcaacaaaaaattgttaatatacctctatactttaacgtcaaggagaaaaaactataatgcaaaaatctcattcagaagaagtgattgtacctgagttcaattctagcgcaaaggaattaccaagaccattggccgaaaagtgcccgagcggtgctnnnnnnnnnnnnnnnnnnnnnnnnnnnnnnnnnnnnnnnnnnnnnnnnnnnnnnnnnnnnnnnnnnnnnnnnnnnnnnnnnnnnnnnnnnnnnnnnnnnnnnnnnnnnnnnnnnnnnnnnnnnnnnnnnnnnnnnnnnnnnnnnnnnnnnnnnnnnnnnnnnnnnnnnnnnnnnnnnnnnnnnnnnnnnnnnnnnnnnnnnnnnnnnnnnnnnnnnnnnnnnnnnnnnnnnnnnnnnnnnnnnnnnnnnnnnnnnnnnnnnnnnnnnnnnnnnnnnnnnnnnnnnnnnnnnnnnnnnnnnnnnnnnnnnnnnnnnnnnnnnnnnnnnnnnnnnnnnnnnnnnnnnnnnnnnnnnnnnnnnnnnnnnnnnnnnnnnnnnnnnnnnnnnnnnnnnnnnnnnnnnnnnnnnnnnnnnnnnnnnnnnnnnnnnnnnnnnnnnnnnnnnnnnnnnnnnnnnnnnnnnnnnnnnnnnnnnnnnnnnnnnnnnnnnnnnnnnnnnnnnnnnnnnnnnnnnnnnnnnnnnnnnnnnnnnnnnnnnnnnnnnnnnnnnnnnnnnnnnnnnnnnnnnnnnnnnnnnnnnnnnnnnnnnnnnnnnnnnnnnnnnnnnnnnnnnnnnnnnnnnnnnnnnnnnnnnnnnnnnnnnnnnnnnnnnnnnnnnnnnnnnnnnnnnnnnnnnnnnnnnnnnnnnnnnnnnnnnnnnnnnnnnnnnnnnnnnnnnnnnnnnnnnnnnnnnnnnnnnnnnnnnnnnnnnnnnnnnnnnnnnnnnnntaatagcatcatgtaattagttatgtcacgcttacattcacgccctccccccacatccgctctaaccgaaaaggaaggagttagacaacctgaagtctaggtccctatttatttttttatagttatgttagtattaagaacgttatttatatttcaaatttttcttttttttctgtacagacgcgtgtacgcatgtaacattatactgaaaaccttgcttgagaaggttttgggacgctcgaaggctttaatttgatacggattagaagccgccgagcgggcgacagccctccgacggaagactctcctccgtgcgtcctcgtcttcaccggtcgcgttcctgaaacgcagatgtgcctcgcgccgcactgctccgaacaataaagattctacaatactagcttttatggttatgaagaggaaaaattggcagtaacctggccccacaaaccttcaaattaacgaatcaaattaacaaccataggatgataatgcgattagttttttagccttatttctggggtaattaatcagcgaagcgatgatttttgatctattaacagatatataaatggaaaagctgcataaccactttaactaatactttcaacattttcagtttgtattacttcttattcaaatgtcataaaagtatcaacaaaaaattgttaatatacctctatactttaacgtcaaggagaaaaaactataatggttaatnnnnnnnnnnnnnnnnnnnnnnnnnnnnnntaatagacaagctacgttgaaacaagaacccgcctcctttcagaactcacttacggtacattagcgatgactacgacttcattactctttttttcagaaaattttaatcaatattcatttattctacgaacagtctccttcaccttagtttctttctctgctcctttgaaactattattgtatttggtacattttagagaaaataaaacatatatagaacaatgagaaggtacgtaatttcttagctaattatttgtaatcaattaagcgtcttcctttagcaaagcgtctctcttttcagcaactctttgagctcttctgtcacgagcagctctgttcttcaatcttctagcttcagcttcttcgttcaaagccttttcacgttgagcatcagccttagcttgaataatgtgttcaaccaaagctctcttgtgcttgaaggcgttacccttggattccttgtacaaaacgtggtacaaatgcttgtcaatcttaccagcgtcacggtacttggccaataatcttctcaagacacgtaatcttctgatccagacgacttgggatggtaaacgagcttctctagtaccctttctcttaccgtaaccactgtgacgaccttctctcttggattgagcatgggctctagttctagatttagagtggacagtaacggccttcttgacgatggttccgttcttgaccaattttctaatggcatttctagagttggcttgggcaatttcagaagtttcgtttgggtctaaccaaacctttctcttaccaacaccgacaacagaagcggcaagtctcttttgagtacgcaagttagccctgtgaaaaaaagtttttgcagatttatttgcatattgatgttagtaaagttgcttcatttttaaaatcctgaaacctaacagtaaagagcatattcgcaaaggttaatgaattactttatctatcaatcgaattaacgcttgcaggaacagacacgtaccattgctgcgataattctatagtttgtaataaacgcggcaattcgtacaagcttgaaatttatctgaggttcttctatggatgttgctaccaactatgcgaccaccggatgctgtatcctcaatttttttccttatctatttctctccaaaggatgacattcataacatatttaaagataaatcttgtgaaaggttcaaaatttagtatcactgttaaacatacattttcctctaatttattggtgactttttattcgatttggtgaaaagatctatcaagtagcactagcgtataaatgtactattagtatcccgatgtagatacagtaagctttggacttcttcgccagaggtttggtcaagtctccaatcaaggttgtcggcttgtctaccttgccagaaatttacgaaaagatggaaaagggtcaaatcgttggtagatacgttgttgacacttctaaataagcgaatttcttatgatttatgatttttattattaaataagttataaaaaaaataagtgtatacaaattttaaagtgactcttaggttttaaaacgaaaattcttattcttgagtaactctttcctgtaggtcaggttgctttctcaggtatagcatgaggtcgctcttattgaccacacctctaccggccggtcgaaattcccctaccctatgaacatattccattttgtaatttcgtgtcgtttctattatgaatttcatttataaagtttatgtacaaatatcataaaaaaagagaatctttttaagcaaggattttcttaacttcttcggcgacagcatcaccgacttcggtggtactgttggaaccacctaaatcaccagttctgatacctgcatccaaaacctttttaactgcatcttcaatggccttaccttcttcaggcaagttcaatgacaatttcaacatcattgcagcagacaagatagtggcgatagggttgaccttattctttggcaaatctggagcagaaccgtggcatggttcgtacaaaccaaatgcggtgttcttgtctggcaaagaggccaaggacgcagatggcaacaaacccaaggaacctgggataacggaggcttcatcggagatgatatcaccaaacatgttgctggtgattataataccatttaggtgggttgggttcttaactaggatcatggcggcagaatcaatcaattgatgttgaaccttcaatgtaggaaattcgttcttgatggtttcctccacagtttttctccataatcttgaagaggccaaaacattagctttatccaaggaccaaataggcaatggtggctcatgttgtagggccatgaaagcggccattcttgtgattctttgcacttctggaacggtgtattgttcactatcccaagcgacaccatcaccatcgtcttcctttctcttaccaaagtaaatacctcccactaattctctgacaacaacgaagtcagtacctttagcaaattgtggcttgattggagataagtctaaaagagagtcggatgcaaagttacatggtcttaagttggcgtacaattgaagttctttacggatttttagtaaaccttgttcaggtctaacactacctgtaccccatttaggaccacccacagcacctaacaaaacggcatcagccttcttggaggcttccagcgcctcatctggaagtgggacacctgtagcttcgatagcagcaccaccaattaaatgattttcgaaatcgaacttgacattggaacgaacatcagaaatagctttaagaaccttaatggcttcggctgtgatttcttgaccaacgtggtcacctggcaaaacgacgatcttcttaggggcagacattagaatggtatatccttgaaatatatatatatattgctgaaatgtaaaaggtaagaaaagttagaaagtaagacgattgctaaccacctattggaaaaaacaataggtccttaaataatattgtcaacttcaagtattgtgatgcaagcatttagtcatgaacgcttctctattctatatgaaaagccggttccggcgctctcacctttcctttttctcccaatttttcagttgaaaaaggtatatgcgtcaggcgacctctgaaattaacaaaaaatttccagtcatcgaatttgattctgtgcgatagcgcccctgtgtgttctcgttatgttgaggaaaaaaataatggttgctaagagattcgaactcttgcatcttacgatacctgagtattcccacagttgggggatctcgactctagctagaggatcaattcgtaatcatgtcatagctgtttcctgtgtgaaattgttatccgctcacaattccacacaacatacgagccggaagcataaagtgtaaagcctggggtgcctaatgagtgagctaactcacattaattgcgttgcgctcactgcccgctttccagtcgggaaacctgtcgtgccagctgataacttcgtataatgtatgctatacgaagttattaggtctgaagaggagtttacgtccagccaagctagcttggctgcaggtcgagcggccgcgatccggaacccttaatataacttcgtataatgtatgctatacgaagttatcagctgcattaatgaatcggccaacgcgcggggagaggcggtttgcgtattgggcgctcttccgcttcctcgctcactgactcgctgcgctcggtcgttcggctgcggcgagcggtatcagctcactcaaaggcggtaatacggttatccacagaatcaggggataacgcaggaaagaacatgtgagcaaaaggccagcaaaaggccaggaaccgtaaaaaggccgcgttgctggcgtttttccataggctccgcccccctgacgagcatcacaaaaatcgacgctcaagtcagaggtggcgaaacccgacaggactataaagataccaggcgtttccccctggaagctccctcgtgcgctctcctgttccgaccctgccgcttaccggatacctgtccgcctttctcccttcgggaagcgtggcgctttctcatagctcacgctgtaggtatctcagttcggtgtaggtcgttcgctccaagctgggctgtgtgcacgaaccccccgttcagcccgaccgctgcgccttatccggtaactatcgtcttgagtccaacccggtaagacacgacttatcgccactggcagcagccactggtaacaggattagcagagcgaggtatgtaggcggtgctacagagttcttgaagtggtggcctaactacggctacactagaagaacagtatttggtatctgcgctctgctgaagccagttaccttcggaaaaagagttggtagctcttgatccggcaaacaaaccaccgctggtagcggtggtttttttgtttgcaagcagcagattacgcgcagaaaaaaaggatctcaagaagatcctttgatcttttctacggggtctgacgctcagtggaacgaaaactcacgttaagggattttggtcatgagattatcaaaaaggatcttcacctagatccttttaaattaaaaatgaagttttaaatcaatctaaagtatatatgagtaaacttggtctgacagttaccaatgcttaatcagtgaggcacctatctcagcgatctgtctatttcgttcatccatagttgcctgactccccgtcgtgtagataactacgatacgggagggcttaccatctggccccagtgctgcaatgataccgcgagacccacgctcaccggctccagatttatcagcaataaaccagccagccggaagggccgagcgcagaagtggtcctgcaactttatccgcctccatccagtctattaattgttgccgggaagctagagtaagtagttcgccagttaatagtttgcgcaacgttgttgccattgctacaggcatcgtggtgtcacgctcgtcgtttggtatggcttcattcagctccggttcccaacgatcaaggcgagttacatgatcccccatgttgtgcaaaaaagcggttagctccttcggtcctccgatcgttgtcagaagtaagttggccgcagtgttatcactcatggttatggcagcactgcataattctcttactgtcatgccatccgtaagatgcttttctgtgactggtgagtactcaaccaagtcattctgagaatagtgtatgcggcgaccgagttgctcttgcccggcgtcaatacgggataataccgcgccacatagcagaactttaaaagtgctcatcattggaaaacgttcttcggggcgaaaactctcaaggatcttaccgctgttgagatccagttcgatgtaacccactcgtgcacccaactgatcttcagcatcttttactttcaccagcgtttctgggtgagcaaaaacaggaaggcaaaatgccgcaaaaaagggaataagggcgacacggaaatgttgaatactcatactcttcctttttcaatattattgaagcatttatcagggttattgtctcatgagcggatacatatttgaatgtatttagaaaaataaacaaataggggttccgcgcacatttccccgaaaagtgccacctgacgtctaagaaaccattattatcatgacattaacctataaaaataggcgtatcacgaggccctttcgtctcgcgcgtttcggtgatgacggtgaaaacctctgacacatgcagctcccggagacggtcacagcttgtctgtaagcggatgccgggagcagacaagcccgtcagggcgcgtcagcgggtgttggcgggtgtcggggctggcttaactatgcggcatcagagcagattgtactgagagtgcaccataacgcatttaagcataaacacgcactatgccgttcttctcatgtatatatatatacaggcaacacgcagatataggtgcgacgtgaacagtgagctgtatgtgcgcagctcgcgttgcattttcggaagcgctcgttttcggaaacgctttgaagttcctattccgaagttcctattctctagctagaaagtataggaacttcagagcgcttttgaaaaccaaaagcgctctgaagacgcactttcaaaaaaccaaaaacgcaccggactgtaacgagctactaaaatattgcgaataccgcttccacaaacattgctcaaaagtatctctttgctatatatctctgtgctatatccctatataacctacccatccacctttcgctccttgaacttgcatctaaactcgacctctacattttttatgtttatctctagtattactctttagacaaaaaaattgtagtaagaactattcatagagtgaatcgaaaacaatacgaaaatgtaaacatttcctatacgtagtatatagagacaaaatagaagaaaccgttcataattttctgaccaatgaagaatcatcaacgctatcactttctgttcacaaagtatgcgcaatccacatcggtatagaatataatcggggatgcctttatcttgaaaaaatgcacccgcagcttcgctagtaatcagtaaacgcgggaagtggagtcaggctttttttatggaagagaaaatagacaccaaagtagccttcttctaaccttaacggacctacagtgcaaaaagttatcaagagactgcattatagagcgcacaaaggagaaaaaaagtaatctaagatgctttgttagaaaaatagcgctctcgggatgcatttttgtagaacaaaaaagaagtatagattctttgttggtaaaatagcgctctcgcgttgcatttctgttctgtaaaaatgcagctcagattctttgtttgaaaaattagcgctctcgcgttgcatttttgttttacaaaaatgaagcacagattcttcgttggtaaaatagcgctttcgcgttgcatttctgttctgtaaaaatgcagctcagattctttgtttgaaaaattagcgctctcgcgttgcatttttgttctacaaaatgaagcacagatgcttcgttgct

SEQ ID NO: 65 - DNA, 7781 bp, synthetic construct
  source 1..7781: mol_type = other DNA
  misc_feature 1..7781: note = Description of Artificial Sequence: Synthetic polynucleotide
cggtgcgggcctcttcgctattacgccagatccttttgttgtttccgggtgtacaatatggacttcctcttttctggcaaccaaacccatacatcgggattcctataataccttcgttggtctccctaacatgtaggtggcggaggggagatatacaatagaacagataccagacaagacataatgggctaaacaagactacaccaattacactgcctcattgatggtggtacataacgaactaatactgtagccctagacttgatagccatcatcatatcgaagtttcactaccctttttccatttgccatctattgaagtaataataggcgcatgcaacttcttttctttttttttcttttctctctcccccgttgttgtctcaccatatccgcaatgacaaaaaaatgatggaagacactaaaggaaaaaattaacgacaaagacagcaccaacagatgtcgttgttccagagctgatgaggggtatctcgaagcacacgaaactttttccttccttcattcacgcacactactctctaatgagcaacggtatacggccttccttccagttacttgaatttgaaataaaaaaaagtttgctgtcttgctatcaagtataaatagacctgcaattattaatcttttgtttcctcgtcattgttctcgttccctttcttccttgtttctttttctgcacaatatttcaagctataccaagcatacaatcaactccaagctttgcaaagatggggtcaaaggccgagctaatcccagagccccctaaaaaaaagagaaaggtcgagctgggaactgcggcagagtacccgtatgatgtaccggactatgccggaggtatgtctagattggacaagtctaaggttatcaactctgctttggaattgttgaacgaagttggtatcgaaggtttgactactagaaagttggctcaaaagttgggtgttgaacaaccaactttgtactggcacgttaagaacaagagagctttgttggacgctttggctatcgaaatgttggacagacaccacactcacttctgtccattggaaggtgaatcttggcaagacttcttgagaaacaacgctaagtctttcagatgtgctttgttgtctcacagagacggtgctaaggttcacttgggtactagaccaactgaaaagcaatacgaaactttggaaaaccaattggctttcttgtgtcaacaaggtttctctttggaaaacgctttgtacgctttgtctgctgttggtcacttcactttgggttgtgttttggaagaccaagaacaccaagttgctaaggaagaaagagaaactccaactactgactctatgccaccattgttgagacaagctatcgaattgttcgaccaccaaggtgctgaaccagctttcttgttcggtttggaattgatcatctgtggtttggaaaagcaattgaagtgtgaatctggttctgggcaaccatctttgagatctgaatacgaatacccagttttctctcacgttcaagctggtatgttctctccagaattgagaactttcactaagggtgacgctgaaagatgggtttctggtccaggtactgaagacgctgaagctgttgctttgggtttgggtttgtctgacttcccatctgctggtaaggctgttttggacgacgaagactctttcgtttggccagctgcttctttcgacatgggtgcttgttgggctggtgctggtttcgctgacccagacccagcttgtatcttcttgaacttgccatgagcccatcttttttttggacctaaattcttcatgaaaatatattacgagggcttattcagaagctttggacttcttcgcttgcagccaagctaattccgggcgaatttcttatgatttatgatttttattattaaataagttataaaaaaaataagtgtatacaaattttaaagtgactcttaggttttaaaacgaaaattcttattcttgagtaactctttcctgtaggtcaggttgctttctcaggtatagcatgaggtcgctcttattgaccacacctctaccggcatgcaagcttggcgtaatcatggtcatagctgtttcctgtgtgaaattgttatccgctcacaattccacacaacatacgagccggaagcataaagtgtaaagcctggggtgcctaatgagtgagctaactcacattaattgcgttgcgctcactgcccgctttccagtcgggaaacctgtcgtgccagctgcattaatgaatcggccaacgcgcggggagaggcggtttgcgtattgggcgctcttccgcttcctcgctcactgactcgctgcgctcggtcgttcggctgcggcgagcggtatcagctcactcaaaggcggtaatacggttatccacagaatcaggggataacgcaggaaagaacatgtgagcaaaaggccagcaaaaggccaggaaccgtaaaaaggccgcgttgctggcgtttttccataggctccgcccccctgacgagcatcacaaaaatcgacgctcaagtcagaggtggcgaaacccgacaggactataaagataccaggcgtttccccctggaagctccctcgtgcgctctcctgttccgaccctgccgcttaccggatacctgtccgcctttctcccttcgggaagcgtggcgctttctcatagctcacgctgtaggtatctcagttcggtgtaggtcgttcgctccaagctgggctgtgtgcacgaaccccccgttcagcccgaccgctgcgccttatccggtaactatcgtcttgagtccaacccggtaagacacgacttatcgccactggcagcagccactggtaacaggattagcagagcgaggtatgtaggcggtgctacagagttcttgaagtggtggcctaactacggctacactagaagaacagtatttggtatctgcgctctgctgaagccagttaccttcggaaaaagagttggtagctcttgatccggcaaacaaaccaccgctggtagcggtggtttttttgtttgcaagcagcagattacgcgcagaaaaaaaggatctcaagaagatcctttgatcttttctacggggtctgacgctcagtggaacgaaaactcacgttaagggattttggtcatgagattatcaaaaaggatcttcacctagatccttttaaattaaaaatgaagttttaaatcaatctaaagtatatatgagtaacctgaggctatggcagggcctgccgccccgacgttggctgcgagccctgggccttcacccgaacttggggggtggggtggggaaaaggaagaaacgcgggcgtattggccccaatggggtctcggtggggtatcgacagagtgccagccctgggaccgaaccccgcgtttatgaacaaacgacccaacaccgtgcgttttattctgtctttttattgccgtcatagcgcgggttccttccggtattgtctccttccgtgtttcagttagcctccccctagggtgggcgaagaactccagcatgagatccccgcgctggaggatcatccagccggcgtcccggaaaacgattccgaagcccaacctttcatagaaggcggcggtggaatcgaaatctcgtgatggcaggttgggcgtcgcttggtcggtcatttcgaaccccagagtcccgctcagaagaactcgtcaagaaggcgatagaaggcgatgcgctgcgaatcgggagcggcgataccgtaaagcacgaggaagcggtcagcccattcgccgccaagctcttcagcaatatcacgggtagccaacgctatgtcctgatagcggtccgccacacccagccggccacagtcgatgaatccagaaaagcggccattttccaccatgatattcggcaagcaggcatcgccatgagtcacgacgagatcctcgccgtcgggcatgctcgccttgagcctggcgaacagttcggctggcgcgagcccctgatgctcttcgtccagatcatcctgatcgacaagaccggcttccatccgagtacgtgctcgctcgatgcgatgtttcgcttggtggtcgaatgggcaggtagccggatcaagcgtatgcagccgccgcattgcatcagccatgatggatactttctcggcaggagcaaggtgagatgacaggagatcctgccccggcacttcgcccaatagcagccagtcccttcccgcttcagtgacaacgtcgagcacagctgcgcaaggaacgcccgtcgtggccagccacgatagccgcgctgcctcgtcttgcagttcattcagggcaccggacaggtcggtcttgacaaaaagaaccgggcgcccctgcgctgacagccggaacacggcggcatcagagcagccgattgtctgttgtgcccagtcatagccgaatagcctctccacccaagcggccggagaacctgcgtgcaatccatcttgttcaatcatactcttcctttttcaatattattgaagcatttatcagggttattgtctcatgagcggatacatatttgaatgtatttagaaaaataaacaaataggggttccgcgcacatttccccgaaaagtgccacctgaacgaagcatctgtgcttcattttgtagaacaaaaatgcaacgcgagagcgctaatttttcaaacaaagaatctgagctgcatttttacagaacagaaatgcaacgcgaaagcgctattttaccaacgaagaatctgtgcttcatttttgtaaaacaaaaatgcaacgcgagagcgctaatttttcaaacaaagaatctgagctgcatttttacagaacagaaatgcaacgcgagagcgctattttaccaacaaagaatctatacttcttttttgttctacaaaaatgcatcccgagagcgctatttttctaacaaagcatcttagattactttttttctcctttgtgcgctctataatgcagtctcttgataactttttgcactgtaggtccgttaaggttagaagaaggctactttggtgtctattttctcttccataaaaaaagcctgactccacttcccgcgtttactgattactagcgaagctgcgggtgcattttttcaagataaaggcatccccgattatattctataccgatgtggattgcgcatactttgtgaacagaaagtgatagcgttgatgattcttcattggtcagaaaattatgaacggtttcttctattttgtctctatatactacgtataggaaatgtttacattttcgtattgttttcgattcactctatgaatagttcttactacaatttttttgtctaaagagtaatactagagataaacataaaaaatgtagaggtcgagtttagatgcaagttcaaggagcgaaaggtggatgggtaggttatatagggatatagcacagagatatatagcaaagagatacttttgagcaatgtttgtggaagcggtattcgcaatattttagtagctcgttacagtccggtgcgtttttggttttttgaaagtgcgtcttcagagcgcttttggttttcaaaagcgctctgaagttcctatactttctagagaataggaacttcggaataggaacttcaaagcgtttccgaaaacgagcgcttccgaaaatgcaacgcgagctgcgcacatacagctcactgttcacgtcgcacctatatctgcgtgttgcctgtatatatatatacatgagaagaacggcatagtgcgtgtttatgcttaaatgcgtacttatatgcgtctatttatgtaggatgaaaggtagtctagtacctcctgtgatattatcccattccatgcggggtatcgtatgcttccttcagcactaccctttagctgttctatatgctgccactcctcaattggattagtctcatccttcaatgctatcatttcctttgatattggatcatactaagaaaccattattatcatgacattaacctataaaaataggcgtatcacgaggccctttcgtctcgcgcgtttcggtgatgacggtgaaaacctctgacacatgcagctcccggagacggtcacagcttgtctgtaagcggatgccgggagcagacaagcccgtcagggcgcgtcagcgggtgttggcgggtgtcggggctggcttaactatgcggcatcagagcagattgtactgagagtgcaccatagatcaacgacattactatatatataatataggaagcatttaatagaacagcatcgtaatatatgtgtactttgcagttatgacgccagatggcagtagtggaagatattctttattgaaaaatagcttgtcaccttacgtacaatcttgatccggagcttttctttttttgccgattaagaattaattcggtcgaaaaaagaaaaggagagggccaagagggagggcattggtgactattgagcacgtgagtatacgtgattaagcacacaaaggcagcttggagtatgtctgttattaatttcacaggtagttctggtccattggtgaaagtttgcggcttgcagagcacagaggccgcagaatgtgctctagattccgatgctgacttgctgggtattatatgtgtgcccaatagaaagagaacaattgacccggttattgcaaggaaaatttcaagtcttgtaaaagcatataaaaatagttcaggcactccgaaatacttggttggcgtgtttcgtaatcaacctaaggaggatgttttggctctggtcaatgattacggcattgatatcgtccaactgcatggagatgagtcgtggcaagaataccaagagttcctcggtttgccagttattaaaagactcgtatttccaaaagactgcaacatactactcagtgcagcttcacagaaacctcattcgtttattcccttgtttgattcagaagcaggtgggacaggtgaacttttggattggaactcgatttctgactgggttggaaggcaagagagccccgaaagcttacattttatgttagctggtggactgacgccagaaaatgttggtgatgcgcttagattaaatggcgttattggtgttgatgtaagcggaggtgtggagacaaatggtgtaaaagactctaacaaaatagcaaatttcgtcaaaaatgctaagaaataggttattactgagtagtatttatttaagtattgtttgtgcacttgccgatctatgcggtgtgaaataccgcacagatgcgtaaggagaaaataccgcatcaggaaattgtaagcgttaatattttgttaaaattcgcgttaaatttttgttaaatcagctcattttttaaccaataggccgaaatcggcaaaatcccttataaatcaaaagaatagaccgagatagggttgagtgttgttccagtttggaacaagagtccactattaaagaacgtggactccaacgtcaaagggcgaaaaaccgtctatcagggcgatggcccactacgtgaaccatcaccctaatcaagttttttggggtcgaggtgccgtaaagcactaaatcggaaccctaaagggagcccccgatttagagcttgacggggaaagccggcgaacgtggcgagaaaggaagggaagaaagcgaaaggagcgggcgctagggcgctggcaagtgtagcggtcacgctgcgcgtaaccaccacacccgccgcgcttaatgcgccgctacagggcgcgtccattcgccattcaggctgcgcaactgttgggaagggcgat

SEQ ID NO: 66 - protein, 20 aa, synthetic construct
  REGION 1..20: note = Description of Artificial Sequence: Synthetic peptide
RRRRRRRKRLGVRLRVSRML

SEQ ID NO: 67 - protein, 27 aa, synthetic construct
  REGION 1..27: note = Description of Artificial Sequence: Synthetic peptide
RQKIWFQNRRMKWKKRLGVRLRVSRML

SEQ ID NO: 68 - protein, 15 aa, synthetic construct
  MOD_RES 2: note = D-2-(7'-octenyl)alanine
  REGION 2..9: note = MISC_FEATURE - Crosslink between residues
  MOD_RES 9: note = 2-(4'-pentenyl)alanine
  REGION 1..15: note = Description of Artificial Sequence: Synthetic peptide
AAKRLGVRARVSRML

SEQ ID NO: 69 - protein, 15 aa, synthetic construct
  REGION 1..15: note = Description of Artificial Sequence: Synthetic peptide
LMRSVRLRVGLRKAG

SEQ ID NO: 70-71 - skipped (2 entries)

SEQ ID NO: 72 - protein, 6 aa, synthetic construct
  MOD_RES 5: note = Met or Val
  MOD_RES 6: note = Leu, Ile, Val, Phe, Met, Ala, Trp or Tyr
  REGION 1..6: note = Description of Artificial Sequence: Synthetic peptide
RLGVXX

SEQ ID NO: 73 - protein, 8 aa, synthetic construct
  REGION 1..2: note = MISC_FEATURE - This region may encompass 1-2 residues
  VARIANT 8: note = X = Leu, Ile, Val, Phe, Met, Ala, Trp or Tyr
  VARIANT 2: note = X = Thr, Lys, Arg or Gln
  VARIANT 7: note = X = Met or Val
  VARIANT 1: note = X = Thr, Lys, Arg or Gln
  REGION 1..8: note = Description of Artificial Sequence: Synthetic peptide
XXRLGVXX

SEQ ID NO: 74-81 - skipped (8 entries)

SEQ ID NO: 82 - protein, 339 aa, Homo sapiens
MAMQMQLEANADTSVEEESFGPQPISRLEQCGINANDVKKLEEAGFHTVEAVAYAPKKELINIKGISEAKADKILAEAAKLVPMGFTTATEFHQRRSEIIQITTGSKELDKLLQGGIETGSITEMFGEFRTGKTQICHTLAVTCQLPIDRGGGEGKAMYIDTEGTFRPERLLAVAERYGLSGSDVLDNVAYARAFNTDHQTQLLYQASAMMVESRYALLIVDSATALYRTDYSGRGELSARQMHLARFLRMLLRLADEFGVAVVITNQVVAQVDGAAMFAADPKKPIGGNIIAHASTTRLYLRKGRGETRICKIYDSPCLPEAEAMFAINADGVGDAKD

SEQ ID NO: 83 - protein, 730 aa, Amanita bisporigera
MPPTPWAPHSYPPTRRSDHVDVYQSASRGEVPVPDPYQWLEENSNEVDEWTTAQTAFTQGYLDKNADRQKLEEKFRASKDYVKFSAPTLLDSGHWYWFYNSGVQSQAVLYRSKKPVLPDFQRGTRKVGEVYFDPNVLSADGTAIMGTCRFSPSGEYFAYAVSHLGVDYFTIYVRPTSSSLSQAPEAEGGDGRLSDGVKWCKFTTITWTKDSKGFLYQRYPARESLVAKDRDKDAMVCYHRVGTTQLEDIIVQQDKENPDWTYGTDASEDGKYIYLVVYKDASKQNLLWVAEFDKDGVKPEIPWRKVINEFGADYHVITNHGSLIYVKTNVNAPQYKVVTIDLSTGEPEIRDFIPEQKDAKLTQVKCVNKGYFVAIYKRNVKDEIYLYSKAGDQLSRLASDFIGVASITNREKQPHSFLTFSGFNTPGTISRYDFTAPDTQRLSILRTTKLNGLNADDFESTQVWYKSKDGTKVPMFIVRHKSTKFDGTAPAIQNGYGGFAITADPFFSPIMLTFMQTYGAILAVPNIRGGGEFGGEWHKAGRRETKGNTFDDFIAAAQFLVKNKYAAPGKVAITGASNGGFLVCGSVVRAPEGTFGAAVSEGGVADLLKFNKFTGGMAWTSEYGNPFIKEDFDFVQALSPVHNVPKDRVLPATLLMTNAGDDRVVPMHSLKFVANLQYNVPQNPHPLLIRVDKSWLGHGFGKTTDKHTKDAADKWSFVAQSLGLEWKTVD

SEQ ID NO: 84 - protein, 730 aa, Galerina marginata
MSSVTWAPGNYPSTRRSDHVDTYQSASKGEVPVPDPYQWLEESTDEVDKWTTAQADLAQSYLDQNADIQKLAEKFRASRNYAKFSAPTLLDDGHWYWFYNRGLQSQSVLYRSNEPALPDFSNGDDNVGDVFFDPNVLATDGSAGMVLCKFSPDGKFFAYAVSHLGGDYSTIYIRSTSSPLSQASAVQGTDGRLSDEVKWFKFSTIIWTKDSKGFLYQRYPARERHEGTRSDRNAMMCYHKVGTTQEEDIIVYQDNEHPEWIYGADTSEDGKYLYLYQFKDTSKKNLLWVAELNEDGVKSGIQWRKVVNEYVADYNVITNHGSLVYIKTNLNAPQYKVITIDLSKDEPEIRDFIPEEKDAKLAQVNCANEEYFVAIYKRNVKDEIYLYSKAGVQLTRLAPDFVGAASIANRQKQTHFFLTLSGFNTPGTIARYDFTAPETQRFSILRTTKVNELDPDDFESTQVWYESKDGTKIPMFIVRHKSTKFDGTAAAIQYGYGGFATSADPFFSPIILTFLQTYGAIFAVPSIRGGGEFGEEWHKGGRRETKVNTFDDFIAAAQFLVKNKYAAPGKVAINGASNGGLLVMGSIVRAPEGTFGAAVPEGGVADLLKFHKFTGGQAWISEYGNPSIPEEFDYIYPLSPVHNVRTDKVMPATLITVNIGDGRVVPMHSFKFIATLQHNVPQNPHPLLIKIDKSWLGHGMGKPTDKNVKDAADKWGFIARALGLELKTVE

SEQ ID NO: 85 - protein, 29 aa, synthetic construct
  MOD_RES 1: note = Lys-(C6-5FAM)
  MOD_RES 1: note = N-terminal Ac
  MOD_RES 29: note = C-terminal NH2
  REGION 1..29: note = Description of Artificial Sequence: Synthetic peptide
KQSLRLGLSRLARVKRLHPGARRRRRRRR

SEQ ID NO: 86 - protein, 29 aa, synthetic construct
  MOD_RES 1: note = Lys-(C6-5FAM)
  MOD_RES 1: note = N-terminal Ac
  MOD_RES 29: note = C-terminal NH2
  REGION 1..29: note = Description of Artificial Sequence: Synthetic peptide
KQSLRLGQSRLARVKRLHPGARRRRRRRR

SEQ ID NO: 87 - protein, 21 aa, synthetic construct
  MOD_RES 1: note = Lys-(C6-5FAM)
  MOD_RES 4: note = NMe-Leu
  MOD_RES 11: note = NMe-Leu
  MOD_RES 14: note = NMe-Val
  MOD_RES 1: note = N-terminal Ac
  MOD_RES 21: note = C-terminal NH2
  REGION 1..21: note = Description of Artificial Sequence: Synthetic peptide
KQSLRLGLSRLARVKRLHPGC

SEQ ID NO: 88 - protein, 9 aa, synthetic construct
  MOD_RES 1: note = N-terminal Ac
  MOD_RES 9: note = C-terminal NH2
  REGION 1..9: note = Description of Artificial Sequence: Synthetic peptide
CRRRRRRRR

SEQ ID NO: 89 - protein, 21 aa, synthetic construct
  MOD_RES 1: note = Lys-(C6-5FAM)
  MOD_RES 1: note = N-terminal Ac
  MOD_RES 21: note = C-terminal NH2
  REGION 1..21: note = Description of Artificial Sequence: Synthetic peptide
KRRRRRRRKRLGVRLRVSRML

SEQ ID NO: 90 - protein, 21 aa, synthetic construct
  MOD_RES 1: note = Lys-(C6-5FAM)
  MOD_RES 1: note = N-terminal Ac
  MOD_RES 21: note = C-terminal NH2
  REGION 1..21: note = Description of Artificial Sequence: Synthetic peptide
KRRRRRRRKRLGQRLRQSRML

SEQ ID NO: 91 - protein, 16 aa, synthetic construct
  MOD_RES 1: note = Lys-(C6-5FAM)
  MOD_RES 1: note = N-terminal Ac
  MOD_RES 16: note = C-terminal NH2
  REGION 1..16: note = Description of Artificial Sequence: Synthetic peptide
KRRRRRRRRLGMSRRF

SEQ ID NO: 92 - protein, 21 aa, synthetic construct
  MOD_RES 1: note = Lys-(C6-5FAM)
  MOD_RES 1: note = N-terminal Ac
  MOD_RES 21: note = C-terminal NH2
  REGION 1..21: note = Description of Artificial Sequence: Synthetic peptide
KRRRRRRRKRLGLRLGVSRRV

SEQ ID NO: 93 - protein, 26 aa, synthetic construct
  MOD_RES 1: note = Lys-(C6-5FAM)
  MOD_RES 1: note = N-terminal Ac
  MOD_RES 26: note = C-terminal NH2
  REGION 1..26: note = Description of Artificial Sequence: Synthetic peptide
KRRRRRRRSLRLGLSRLARVKRLHPG

SEQ ID NO: 94 - protein, 20 aa, synthetic construct
  MOD_RES 1: note = N-terminal Ac
  MOD_RES 20: note = C-terminal NH2
  REGION 1..20: note = Description of Artificial Sequence: Synthetic peptide
RRRRRRRKRLGVRLRVSRML

SEQ ID NO: 95 - protein, 27 aa, synthetic construct
  MOD_RES 1: note = N-terminal Ac
  MOD_RES 27: note = C-terminal NH2
  REGION 1..27: note = Description of Artificial Sequence: Synthetic peptide
RQKIWFQNRRMKWKKRLGVRLRVSRML

SEQ ID NO: 96 - protein, 15 aa, synthetic construct
  MOD_RES 2: note = D-2-(7'-octenyl)alanine
  REGION 2..9: note = MISC_FEATURE - Crosslink between residues
  MOD_RES 9: note = 2-(4'-pentenyl)alanine
  MOD_RES 1: note = N-terminal Ac
  MOD_RES 15: note = C-terminal NH2
  REGION 1..15: note = Description of Artificial Sequence: Synthetic peptide
AAKRLGVRARVSRML

SEQ ID NO: 97 - protein, 24 aa, synthetic construct
  REGION 1..24: note = Description of Artificial Sequence: Synthetic peptide
KGDAERWVSGPGAPLLNKRISYDL

SEQ ID NO: 98 - protein, 37 aa, synthetic construct
  REGION 1..37: note = Description of Artificial Sequence: Synthetic polypeptide
EQKLISEEDLFKPGGGSGPGTEDAEAVALGLGLSDFP

SEQ ID NO: 99 - protein, 15 aa, synthetic construct
  REGION 1..15: note = Description of Artificial Sequence: Synthetic peptide
TSYVETRTRLLSELT

SEQ ID NO: 100 - protein, 29 aa, synthetic construct
  MOD_RES 1: note = Lys-(C6-5FAM)
  MOD_RES 4: note = NMe-Leu
  MOD_RES 11: note = NMe-Leu
  MOD_RES 14: note = NMe-Val
  MOD_RES 1: note = N-terminal Ac
  MOD_RES 29: note = C-terminal NH2
  REGION 1..29: note = Description of Artificial Sequence: Synthetic polypeptide
KQSLRLGLSRLARVKRLHPGARRRRRRRR

SEQ ID NO: 101 - protein, 87 aa, Homo sapiens
YIDTEGTFRPERLLAVAERYGLSGSDVLDNVAYARAFNTDHQTQLLYQASAMMVESRYALLIVDSATALYRTDYSGRGELSARQMHL

SEQ ID NO: 102 - protein, 87 aa, Gallus gallus
YIDTEGTFRPERLLAVAERYGLSGSDVLDNVAYARGFNTDHQTQLLYQASAMMAESRYALLIVDSATALYRTDYSGRGELSARQMHL

SEQ ID NO: 103 - protein, 87 aa, Danio rerio
YIDTEGTFRPERLLAVAERYGLVGSDVLDNVAYARAFNTDHQTQLLYQASAMMTESRYALLIVDSATALYRTDYSGRGELSARQGHL

SEQ ID NO: 104 - protein, 87 aa, Xenopus laevis
YIDTEGTFRPERLLAVAERYGLSGSDVLDNVAYARAFNTDHQTQLLYQASAMMAESRYALLIVDSATALYRTDYSGRGELSARQMHL

SEQ ID NO: 105 - protein, 87 aa, Ustilago maydis
YIDTENTFRPTRLLAVAERFGLNGEEVLDNVAYARAYNADHQLQLLMQASAMMAESRFSLLIVDSLTSLYRTDFSGRGELSARQMHL

SEQ ID NO: 106 - protein, 87 aa, Schizosaccharomyces pombe
YIDTEGTFRPVRLLAVADRYGLNGEEVLDNVAYARAYNADHQLELLQQAANMMSESRFSLLVVDSCTALYRTDFSGRGELSARQMHL

SEQ ID NO: 107 - protein, 87 aa, Schizosaccharomyces japonicus
YIDTEGTFRPVRLLAVAERYGLNGEEVLDNVAYARAYNADHQLELLQQAANMMAESRFSLLVVDSCTALYRTDFSGRGELSARQMHL

SEQ ID NO: 108 - protein, 87 aa, Pichia membranifaciens
FIDTESTFRPIRIVPIARRFGLDEHEAMENIAYARAYNADHQLQLLNQAAQMMAQSRFSLLVVDSIMALYRTDYSGRGELSARQMHV

SEQ ID NO: 109 - protein, 87 aa, Pichia kudriavzevii
FIDTESTFRPVRIVPIARRFGLDEREAMENIAYARAYNADHQLQLLNQAAQMMAQSRFSLLIVDSIMALYRTDYSGRGELSARQMHV

SEQ ID NO: 110 - protein, 87 aa, Arthrobotrys oligospora
YIDTEGTFRPVRLLAVAQRYGLNGEEVLDNVAYARAYNSDHQLQLLNMAAQMMTETRFSLLIVDSATSLYRTDFSGRGDLSARQMHL

SEQ ID NO: 111 - protein, 87 aa, Dactylellina haptotyla
YIDTEGTFRPVRLVSIAQRYGLNPEDCLDNVAYARAYNAEHQFQLLNHAAQMMSESRFSCLIVDSIMSLYRTDYSGRAELSARQTHV

SEQ ID NO: 112 - protein, 87 aa, Millerozyma farinose
YIDTEGTFRPVRLVSIAQRYGLNPDDCLDNVAYARAYNADHQFQLLNLAAQMMAESRFSLLIVDSIMSLYRTDYSGRGELSARQSHV

SEQ ID NO: 113 - protein, 87 aa, Debaryomyces hansenii; identical to SEQ ID NO: 111

SEQ ID NO: 114 - protein, 87 aa, Ogataea parapolymorpha
YIDTEGTFRPIRLVAIARRFGLDENETLDNVAYARAYNADHQLQLLHQAASMMTESRFSLLIVDSIMALYRTDYSGRGELSARQMHV

SEQ ID NO: 115 - protein, 87 aa, Komagataella phaffii
YIDTEGTFRPIRLVSIAKRYGLNEDDTLDNVAYARAYNADHQLQLLNQAAAMMSESRFSLLIVDSIMALYRTDFSGRGELSARQMHV

SEQ ID NO: 116 - protein, 87 aa, Aspergillus clavatus
YIDTEGTFRPVRLLAVAQRYGLVGEEVLDNVAYARAYNSDHQLQLLNQASQMMCETRFSLLVVDSATSLYRTDFNGRGELSSRQTHL

SEQ ID NO: 117 - protein, 87 aa, Pneumocystis jirovecii
YIDTEGTFRPTRLLAVADRYGLNGEEVLDNVAYARAYNADHQLQLLGQAANMMAESRFSLLIVDSATSLYRTDFAGRGELSARQMHL

SEQ ID NO: 118 - protein, 87 aa, Yarrowia lipolytica
YIDTEGTFRPERLHQIARRYGLNGDEVLDNVAYARAHNSDHQMQLLQMAANMMTKSRFSCLIVDSIMALYRTDYAGRGELSARQTHV

SEQ ID NO: 119 - protein, 87 aa, Candida albicans
YIDTEGTFRPNRLVSIAQRYGLNPNDCLDNVAYARAYNAEHQLNLLNIAAEMMAESRFSLLIVDSIMSLYRTDYAGRGELSARQTHV

SEQ ID NO: 120 - protein, 87 aa, Wickerhamomyces ciferrii
YIDTEGTFRPVRLVSIARRYGLNEDDALDNVAYARAYNADHQLQLLNQAAAMMSESRFSLLIVDSIMALYRTDFAGRGELSARQMHV

SEQ ID NO: 121 - protein, 87 aa, Cyberlindnera fabianii
YIDTEGTFRPVRLVSIARRYGLNEDDALDNVAYARAYNADHQLSLLNQAAAMMSESRFSLLIVDSIMALYRTDFAGRGELSARQMHV

SEQ ID NO: 122 - protein, 87 aa, Candida dubliniensis
YIDTEGTFRPNRLVSIAQRYGLNPNDCLDNVAYARAYNAEHQLNLLNIASQMMAESRFSLLIVDSIMSLYRTDYAGRGELSARQTHV

SEQ ID NO: 123 - protein, 87 aa, Lodderomyces elongisporus
YIDTEGTFRPNRLVSIAERYGLNANDCLDNVAYARAYNAEHQLNLLNLAAEMMAESRFSLLIVDSIMSLYRTDYAGRGELSARQTSV

SEQ ID NO: 124 - protein, 87 aa, Candida maltosa
YIDTEGTFRPNRLISIAERYGLNPNDCLDNVAYARAYNAEHQLNLLNVAAQMMAESRFSLLIVDSIMSLYRTDYAGRGELSARQTHV

SEQ ID NO: 125 - protein, 87 aa, Candida tropicalis
YIDTEGTFRPNRLISIAERYGLNANDCLDNVAYARAYNAEHQLNLLNIAAQMMAESRFSLLIVDSIMSLYRTDYAGRGELSARQTHV

SEQ ID NO: 126 - protein, 87 aa, Zygosaccharomyces bailii
YIDTEGTFRPVRLVSIAQRFGLDPDDALNNVAYARAYNADHQIRLLDAAAQMMSESRFSLVVVDSVMALYRTDFSGRGELSARQMHL

SEQ ID NO: 127 - protein, 87 aa, Lachancea mirantina
YIDTEGTFRPIRLVSIAQRFGLDPDDALNNVAYARAYNADHQLRLLDAAAQMMSESRFSLIVVDSIMALYRTDFSGRGELSARQMHL

SEQ ID NO: 128 - protein, 87 aa, Candida glabrata
YIDTEGTFRPVRLVSIAQRFGLDPDDALNNVAYARAYNADHQMRLLDAAAQMMSESRFSLIVVDSVMALYRTDFSGRGELSARQMHL

SEQ ID NO: 129 - protein, 87 aa, Kazachstania saulgeensis
YIDTEGTFRPIRLVSIAQRFGLDPDDALNNVAYARAYNADHQLKLLDAAAQMMSESRFSLIVVDSVMALYRTDFSGRGELSARQMHL

SEQ ID NO: 130 - protein, 87 aa, Naumovozyma dairenensis
YIDTEGTFRPVRLVSIAQRFGLDPDDALNNVAYARAYNADHQLKLLDAASQMMSESRFSLIIVDSVMALYRTDFSGRGELSARQMHL

SEQ ID NO: 131 - protein, 87 aa, Kluyveromyces lactis
YIDTEGTFRPIRLVSIAQRFGLDPDDALNNVAYARAYNADHQLKLLDAAAQMMSESRFSLIIVDSIMALYRTDFSGRGELSARQMHL

SEQ ID NO: 132 - protein, 87 aa, Kluyveromyces dobzhanskii; identical to SEQ ID NO: 131

SEQ ID NO: 133 - protein, 87 aa, Zygosaccharomyces rouxii; identical to SEQ ID NO: 126

SEQ ID NO: 134 - protein, 87 aa, Naumovozyma castelli
YIDTEGTFRPVRLVSIAQRFGLDPDDALNNVAYARAYNADHQLRLLDAAAQMMSESRFSLIIVDSVMALYRTDFSGRGELSARQMHL

SEQ ID NO: 135 - protein, 87 aa, Torulaspora delbrueckii
YIDTEGTFRPVRLVSIAQRFGLDPDDALNNVAYARAYNADHQIRLLDAAAQMMSESRFSLIVVDSVMALYRTDFSGRGELSARQMHL

SEQ ID NO: 136 - protein, 87 aa, Lachancea dasiensis
YIDTEGTFRPIRLVSIAQRFGLDPDDALNNVAYARAYNADHQLRLLDAAAQMMSESRFSLIVVDSIMALYRTDFAGRGELSARQMHL

SEQ ID NO: 137 - protein, 87 aa, Kazachstania africana
YIDTEGTFRPIRLVSIAQRFGLDPDDALNNVAYARAYNADHQLRLLDAAAQMMSESRFSLIIVDSVMALYRTDFSGRGELSARQMHL

SEQ ID NO: 138 - protein, 87 aa, Eremothecium sinecaudum; identical to SEQ ID NO: 127

SEQ ID NO: 139 - protein, 87 aa, Ashbya aceri; identical to SEQ ID NO: 127

SEQ ID NO: 140 - protein, 87 aa, Vanderwaltozyma polyspora; identical to SEQ ID NO: 135

SEQ ID NO: 141 - protein, 87 aa, Eremothecium gossypii; identical to SEQ ID NO: 127

SEQ ID NO: 142 - protein, 87 aa, Lachancea nothofagi
YIDTEGTFRPIRLVSIAQRFGLDPDDALNNVAYARAYNADHQLRLLDAAAQMMSESRFSVIVVDSIMALYRTDFSGRGELSARQMHL

SEQ ID NO: 143 - protein, 87 aa, Eremothecium cymbalariae; identical to SEQ ID NO: 127

SEQ ID NO: 144 - protein, 87 aa, Saccharomyces cerevisiae
YIDTEGTFRPVRLVSIAQRFGLDPDDALNNVAYARAYNADHQLRLLDAAAQMMSESRFSLIVVDSVMALYRTDFSGRGELSARQMHL